European Patent Specification EP 3 615 574 B1, published June 24, 2026. Title: CONSTRUCTS SPECIFICALLY RECOGNIZING GLYPICAN 3 AND USES THEREOF. Applicant: Eureka Therapeutics, Inc. Zhang, Pengbo Xu, Yiyang Morales, Javier Nakano, Yoko Liu, Hong Xiang, Jingyi Acker, Timothy. Application Not Yet Assigned. The sequence listing filed with the application follows.

SEQUENCE LISTING (536 sequences)

SEQ ID NO: 1 - protein, 8 aa, Artificial Sequence
  GPC3A-034 HCDR1
GGSFSGYY

SEQ ID NO: 2 - protein, 8 aa, Artificial Sequence
  GPC3A-035 HCDR1
GYTFTGYY

SEQ ID NO: 3 - protein, 8 aa, Artificial Sequence
  GPC3A-037 HCDR1
GFTFSSYA

SEQ ID NO: 4 - protein, 8 aa, Artificial Sequence
  GPC3A-038 HCDR1
GYTFTSYY

SEQ ID NO: 5 - protein, 8 aa, Artificial Sequence
  GPC3A-039 HCDR1
GFTFSSYA

SEQ ID NO: 6 - protein, 8 aa, Artificial Sequence
  GPC3A-040 HCDR1
GYTFTGYY

SEQ ID NO: 7 - protein, 8 aa, Artificial Sequence
  GPC3A-041 HCDR1
GYTFTGYY

SEQ ID NO: 8 - protein, 8 aa, Artificial Sequence
  GPC3A-042 HCDR1
GYSFTGYY

SEQ ID NO: 9 - protein, 8 aa, Artificial Sequence
  GPC3A-043 HCDR1
GYTFTDYY

SEQ ID NO: 10 - protein, 8 aa, Artificial Sequence
  GPC3A-044 HCDR1
GGSFSGYY

SEQ ID NO: 11 - protein, 8 aa, Artificial Sequence
  GPC3A-045 HCDR1
GFTFSDYY

SEQ ID NO: 12 - protein, 8 aa, Artificial Sequence
  GPC3A-046 HCDR1
GYRFSNYG

SEQ ID NO: 13 - protein, 8 aa, Artificial Sequence
  GPC3A-047 HCDR1
GYTFTGYY

SEQ ID NO: 14 - protein, 8 aa, Artificial Sequence
  GPC3A-048 HCDR1
GFTFSSYA

SEQ ID NO: 15 - protein, 8 aa, Artificial Sequence
  GPC3A-049 HCDR1
GYTFTGYY

SEQ ID NO: 16 - protein, 8 aa, Artificial Sequence
  GPC3A-050 HCDR1
GYSFTGYY

SEQ ID NO: 17 - protein, 8 aa, Artificial Sequence
  GPC3A-051 HCDR1
GGAFSSYA

SEQ ID NO: 18 - protein, 8 aa, Artificial Sequence
  GPC3A-052 HCDR1
GYTFTGYY

SEQ ID NO: 19 - protein, 10 aa, Artificial Sequence
  GPC3A-053 HCDR1
GGSISSSSYY

SEQ ID NO: 20 - protein, 8 aa, Artificial Sequence
  GPC3A-054 HCDR1
GYTFTSYG

SEQ ID NO: 21 - protein, 8 aa, Artificial Sequence
  GPC3A-055 HCDR1
GYTFTSYY

SEQ ID NO: 22 - protein, 8 aa, Artificial Sequence
  GPC3A-056 HCDR1
GYSFNDYY

SEQ ID NO: 23 - protein, 8 aa, Artificial Sequence
  GPC3A-057 HCDR1
GFTFSSYA

SEQ ID NO: 24 - protein, 8 aa, Artificial Sequence
  GPC3A-058 HCDR1
GYTFASHG

SEQ ID NO: 25 - protein, 8 aa, Artificial Sequence
  GPC3A-059 HCDR1
GYTFTRYG

SEQ ID NO: 26 - protein, 8 aa, Artificial Sequence
  GPC3A-060 HCDR1
GYTFNSYA

SEQ ID NO: 27 - protein, 8 aa, Artificial Sequence
  GPC3A-061 HCDR1
GYTFTSYG

SEQ ID NO: 28 - protein, 8 aa, Artificial Sequence
  GPC3A-062 HCDR1
GGTFSSYA

SEQ ID NO: 29 - protein, 8 aa, Artificial Sequence
  GPC3A-063 HCDR1
GYTFTSYY

SEQ ID NO: 30 - protein, 8 aa, Artificial Sequence
  GPC3A-064 HCDR1
GYTFTIYG

SEQ ID NO: 31 - protein, 8 aa, Artificial Sequence
  GPC3A-067 HCDR1
GGTFSSYA

SEQ ID NO: 32 - protein, 8 aa, Artificial Sequence
  GPC3B-54 HCDR1
GYTFIDYY

SEQ ID NO: 33 - protein, 8 aa, Artificial Sequence
  GPC3B-60 HCDR1
GYTFTSYY

SEQ ID NO: 34 - protein, 8 aa, Artificial Sequence
  GPC3B-63 HCDR1
GYTFTSYY

SEQ ID NO: 35 - protein, 8 aa, Artificial Sequence
  GPC3B-66 HCDR1
GYTFIGQY

SEQ ID NO: 36 - protein, 8 aa, Artificial Sequence
  GPC3B-68 HCDR1
GGTFSSYA

SEQ ID NO: 37 - protein, 8 aa, Artificial Sequence
  GPC3B-71 HCDR1
GFTFSRYT

SEQ ID NO: 38 - protein, 8 aa, Artificial Sequence
  GPC3B-76 HCDR1
GYTFTDYY

SEQ ID NO: 39 - protein, 8 aa, Artificial Sequence
  GPC3B-78 HCDR1
GYTFTSYY

SEQ ID NO: 40 - protein, 8 aa, Artificial Sequence
  GPC3B-80 HCDR1
GGTLSRFA

SEQ ID NO: 41 - protein, 8 aa, Artificial Sequence
  GPC3B-81 HCDR1
GYTFTGYY

SEQ ID NO: 42 - protein, 8 aa, Artificial Sequence
  GPC3B-82 HCDR1
GYSFTSYY

SEQ ID NO: 43 - protein, 8 aa, Artificial Sequence
  GPC3B-85 HCDR1
GYTFTSYA

SEQ ID NO: 44 - protein, 8 aa, Artificial Sequence
  GPC3B-87 HCDR1
GGTFGSYA

SEQ ID NO: 45 - protein, 8 aa, Artificial Sequence
  GPC3B-92 HCDR1
GYTFSNYY

SEQ ID NO: 46 - protein, 8 aa, Artificial Sequence
  GPC3B-93 HCDR1
GYTFTSYY

SEQ ID NO: 47 - protein, 8 aa, Artificial Sequence
  GPC3B-110 HCDR1
GGTFTTYS

SEQ ID NO: 48 - protein, 8 aa, Artificial Sequence
  GPC3B-113 HCDR1
GYTLTELS

SEQ ID NO: 49 - protein, 8 aa, Artificial Sequence
  GPC3B-115 HCDR1
GYTFTAYY

SEQ ID NO: 50 - protein, 8 aa, Artificial Sequence
  GPC3B-119 HCDR1
GYTFTSYA

SEQ ID NO: 51 - protein, 8 aa, Artificial Sequence
  GPC3B-125 HCDR1
GYTFTSYA

SEQ ID NO: 52 - protein, 7 aa, Artificial Sequence
  GPC3A-034 HCDR2
INHSGST

SEQ ID NO: 53 - protein, 8 aa, Artificial Sequence
  GPC3A-035 HCDR2
INPNSGGT

SEQ ID NO: 54 - protein, 8 aa, Artificial Sequence
  GPC3A-037 HCDR2
IYSGGSST

SEQ ID NO: 55 - protein, 8 aa, Artificial Sequence
  GPC3A-038 HCDR2
INPSGGST

SEQ ID NO: 56 - protein, 7 aa, Artificial Sequence
  GPC3A-039 HCDR2
IGTGGGT

SEQ ID NO: 57 - protein, 8 aa, Artificial Sequence
  GPC3A-040 HCDR2
INPNSGGT

SEQ ID NO: 58 - protein, 8 aa, Artificial Sequence
  GPC3A-041 HCDR2
INPNSGGT

SEQ ID NO: 59 - protein, 8 aa, Artificial Sequence
  GPC3A-042 HCDR2
MNPRSGGT

SEQ ID NO: 60 - protein, 8 aa, Artificial Sequence
  GPC3A-043 HCDR2
VDPEDGET

SEQ ID NO: 61 - protein, 7 aa, Artificial Sequence
  GPC3A-044 HCDR2
INHSGST

SEQ ID NO: 62 - protein, 8 aa, Artificial Sequence
  GPC3A-045 HCDR2
ISSSGSTI

SEQ ID NO: 63 - protein, 8 aa, Artificial Sequence
  GPC3A-046 HCDR2
ISGSNGNT

SEQ ID NO: 64 - protein, 8 aa, Artificial Sequence
  GPC3A-047 HCDR2
INPNSGGT

SEQ ID NO: 65 - protein, 8 aa, Artificial Sequence
  GPC3A-048 HCDR2
ISYDGSNK

SEQ ID NO: 66 - protein, 8 aa, Artificial Sequence
  GPC3A-049 HCDR2
INPNSGGT

SEQ ID NO: 67 - protein, 8 aa, Artificial Sequence
  GPC3A-050 HCDR2
MNPRSGGT

SEQ ID NO: 68 - protein, 8 aa, Artificial Sequence
  GPC3A-051 HCDR2
IIPIFGTA

SEQ ID NO: 69 - protein, 8 aa, Artificial Sequence
  GPC3A-052 HCDR2
INPNSGGT

SEQ ID NO: 70 - protein, 7 aa, Artificial Sequence
  GPC3A-053 HCDR2
IYYSGST

SEQ ID NO: 71 - protein, 8 aa, Artificial Sequence
  GPC3A-054 HCDR2
ISAYNGNT

SEQ ID NO: 72 - protein, 8 aa, Artificial Sequence
  GPC3A-055 HCDR2
INPSGGST

SEQ ID NO: 73 - protein, 8 aa, Artificial Sequence
  GPC3A-056 HCDR2
INPNNGDT

SEQ ID NO: 74 - protein, 8 aa, Artificial Sequence
  GPC3A-057 HCDR2
ISGSGGST

SEQ ID NO: 75 - protein, 8 aa, Artificial Sequence
  GPC3A-058 HCDR2
ISPYTGNT

SEQ ID NO: 76 - protein, 8 aa, Artificial Sequence
  GPC3A-059 HCDR2
ISAYSDKT

SEQ ID NO: 77 - protein, 8 aa, Artificial Sequence
  GPC3A-060 HCDR2
ISAYNGNT

SEQ ID NO: 78 - protein, 8 aa, Artificial Sequence
  GPC3A-061 HCDR2
ISAYNGNT

SEQ ID NO: 79 - protein, 8 aa, Artificial Sequence
  GPC3A-062 HCDR2
IIPKIGTA

SEQ ID NO: 80 - protein, 8 aa, Artificial Sequence
  GPC3A-063 HCDR2
INPSGGSA

SEQ ID NO: 81 - protein, 8 aa, Artificial Sequence
  GPC3A-064 HCDR2
ISPYNDNT

SEQ ID NO: 82 - protein, 8 aa, Artificial Sequence
  GPC3A-067 HCDR2
IIPIFGIT

SEQ ID NO: 83 - protein, 8 aa, Artificial Sequence
  GPC3B-54 HCDR2
IIPIFGTA

SEQ ID NO: 84 - protein, 8 aa, Artificial Sequence
  GPC3B-60 HCDR2
INPSGGST

SEQ ID NO: 85 - protein, 8 aa, Artificial Sequence
  GPC3B-63 HCDR2
INPSGGST

SEQ ID NO: 86 - protein, 8 aa, Artificial Sequence
  GPC3B-66 HCDR2
INPMTGVT

SEQ ID NO: 87 - protein, 8 aa, Artificial Sequence
  GPC3B-68 HCDR2
IIPILGIA

SEQ ID NO: 88 - protein, 8 aa, Artificial Sequence
  GPC3B-71 HCDR2
ISSSGSYI

SEQ ID NO: 89 - protein, 8 aa, Artificial Sequence
  GPC3B-76 HCDR2
INPNSGGT

SEQ ID NO: 90 - protein, 8 aa, Artificial Sequence
  GPC3B-78 HCDR2
INPSGGST

SEQ ID NO: 91 - protein, 8 aa, Artificial Sequence
  GPC3B-80 HCDR2
IIPIFRTA

SEQ ID NO: 92 - protein, 8 aa, Artificial Sequence
  GPC3B-81 HCDR2
INPNSGGT

SEQ ID NO: 93 - protein, 8 aa, Artificial Sequence
  GPC3B-82 HCDR2
INPSGGST

SEQ ID NO: 94 - protein, 8 aa, Artificial Sequence
  GPC3B-85 HCDR2
INTNTGNP

SEQ ID NO: 95 - protein, 8 aa, Artificial Sequence
  GPC3B-87 HCDR2
IIPVLGRT

SEQ ID NO: 96 - protein, 8 aa, Artificial Sequence
  GPC3B-92 HCDR2
INPSGGTT

SEQ ID NO: 97 - protein, 8 aa, Artificial Sequence
  GPC3B-93 HCDR2
INPSGGST

SEQ ID NO: 98 - protein, 8 aa, Artificial Sequence
  GPC3B-110 HCDR2
IIPTFGTT

SEQ ID NO: 99 - protein, 8 aa, Artificial Sequence
  GPC3B-113 HCDR2
FDPEDGET

SEQ ID NO: 100 - protein, 8 aa, Artificial Sequence
  GPC3B-115 HCDR2
INANTGGT

SEQ ID NO: 101 - protein, 8 aa, Artificial Sequence
  GPC3B-119 HCDR2
INTNTGNP

SEQ ID NO: 102 - protein, 8 aa, Artificial Sequence
  GPC3B-125 HCDR2
INTNTGNP

SEQ ID NO: 103 - protein, 10 aa, Artificial Sequence
  GPC3A-034 HCDR3
ARGYGGRFDY

SEQ ID NO: 104 - protein, 10 aa, Artificial Sequence
  GPC3A-035 HCDR3
ARSWTSGFDY

SEQ ID NO: 105 - protein, 11 aa, Artificial Sequence
  GPC3A-037 HCDR3
ARTSYLNHGDY

SEQ ID NO: 106 - protein, 9 aa, Artificial Sequence
  GPC3A-038 HCDR3
ARKVTGYDS

SEQ ID NO: 107 - protein, 10 aa, Artificial Sequence
  GPC3A-039 HCDR3
ARYGRKSIDA

SEQ ID NO: 108 - protein, 10 aa, Artificial Sequence
  GPC3A-040 HCDR3
ARRGYYGYDS

SEQ ID NO: 109 - protein, 10 aa, Artificial Sequence
  GPC3A-041 HCDR3
ARSGKYYGDK

SEQ ID NO: 110 - protein, 10 aa, Artificial Sequence
  GPC3A-042 HCDR3
ARSSYYWADS

SEQ ID NO: 111 - protein, 17 aa, Artificial Sequence
  GPC3A-043 HCDR3
ARELRDVAYYPWGVEDF

SEQ ID NO: 112 - protein, 10 aa, Artificial Sequence
  GPC3A-044 HCDR3
ARYYVPYLSD

SEQ ID NO: 113 - protein, 9 aa, Artificial Sequence
  GPC3A-045 HCDR3
ARASDLYGD

SEQ ID NO: 114 - protein, 14 aa, Artificial Sequence
  GPC3A-046 HCDR3
ARGNRRYYSPIIDP

SEQ ID NO: 115 - protein, 11 aa, Artificial Sequence
  GPC3A-047 HCDR3
ARSDYGSLYDK

SEQ ID NO: 116 - protein, 10 aa, Artificial Sequence
  GPC3A-048 HCDR3
ARSSFVATDY

SEQ ID NO: 117 - protein, 14 aa, Artificial Sequence
  GPC3A-049 HCDR3
ARHGGIGSMRSFDQ

SEQ ID NO: 118 - protein, 10 aa, Artificial Sequence
  GPC3A-050 HCDR3
ARSGYRWLDV

SEQ ID NO: 119 - protein, 14 aa, Artificial Sequence
  GPC3A-051 HCDR3
ARMLYLSGRYYWDS

SEQ ID NO: 120 - protein, 10 aa, Artificial Sequence
  GPC3A-052 HCDR3
ARSHSSGYDK

SEQ ID NO: 121 - protein, 10 aa, Artificial Sequence
  GPC3A-053 HCDR3
ARWWSGSYDT

SEQ ID NO: 122 - protein, 12 aa, Artificial Sequence
  GPC3A-054 HCDR3
ARIPMYSGSSDY

SEQ ID NO: 123 - protein, 10 aa, Artificial Sequence
  GPC3A-055 HCDR3
ARWHGGPYDY

SEQ ID NO: 124 - protein, 15 aa, Artificial Sequence
  GPC3A-056 HCDR3
ARFSTHNWWWPTYDY

SEQ ID NO: 125 - protein, 13 aa, Artificial Sequence
  GPC3A-057 HCDR3
ARYNYMSSGFYDR

SEQ ID NO: 126 - protein, 13 aa, Artificial Sequence
  GPC3A-058 HCDR3
ARGKRTLASCFDY

SEQ ID NO: 127 - protein, 10 aa, Artificial Sequence
  GPC3A-059 HCDR3
ARSRWSYMDV

SEQ ID NO: 128 - protein, 12 aa, Artificial Sequence
  GPC3A-060 HCDR3
AREGYGSWAMDQ

SEQ ID NO: 129 - protein, 10 aa, Artificial Sequence
  GPC3A-061 HCDR3
ARKGSSQFDQ

SEQ ID NO: 130 - protein, 16 aa, Artificial Sequence
  GPC3A-062 HCDR3
ARMYMDMGWGWGYWDW

SEQ ID NO: 131 - protein, 12 aa, Artificial Sequence
  GPC3A-063 HCDR3
ARDRLASDAFDI

SEQ ID NO: 132 - protein, 13 aa, Artificial Sequence
  GPC3A-064 HCDR3
ARMGVGWGYAQDS

SEQ ID NO: 133 - protein, 9 aa, Artificial Sequence
  GPC3A-067 HCDR3
ARGAEMSDY

SEQ ID NO: 134 - protein, 13 aa, Artificial Sequence
  GPC3B-54 HCDR3
ARERRYSSSPSDH

SEQ ID NO: 135 - protein, 12 aa, Artificial Sequence
  GPC3B-60 HCDR3
ARSLYSQPYIDG

SEQ ID NO: 136 - protein, 15 aa, Artificial Sequence
  GPC3B-63 HCDR3
ARSLHAMRWSQTMDS

SEQ ID NO: 137 - protein, 11 aa, Artificial Sequence
  GPC3B-66 HCDR3
ARFSSGYSRDT

SEQ ID NO: 138 - protein, 10 aa, Artificial Sequence
  GPC3B-68 HCDR3
ARYGYEGHDT

SEQ ID NO: 139 - protein, 13 aa, Artificial Sequence
  GPC3B-71 HCDR3
ARQGHMWYVPVDA

SEQ ID NO: 140 - protein, 5 aa, Artificial Sequence
  GPC3B-76 HCDR3
ARNYD

SEQ ID NO: 141 - protein, 10 aa, Artificial Sequence
  GPC3B-78 HCDR3
ARGYSSFFDS

SEQ ID NO: 142 - protein, 15 aa, Artificial Sequence
  GPC3B-80 HCDR3
ARMSKYYGSYSSYDE

SEQ ID NO: 143 - protein, 7 aa, Artificial Sequence
  GPC3B-81 HCDR3
ARGLWDS

SEQ ID NO: 144 - protein, 14 aa, Artificial Sequence
  GPC3B-82 HCDR3
ARYPVYMETSDFDS

SEQ ID NO: 145 - protein, 18 aa, Artificial Sequence
  GPC3B-85 HCDR3
ARSSLYWMGSKWSRQTDM

SEQ ID NO: 146 - protein, 6 aa, Artificial Sequence
  GPC3B-87 HCDR3
ARTNDS

SEQ ID NO: 147 - protein, 13 aa, Artificial Sequence
  GPC3B-92 HCDR3
ARPSMWTSSMGDV

SEQ ID NO: 148 - protein, 16 aa, Artificial Sequence
  GPC3B-93 HCDR3
ARYTALKPRGIYSVDS

SEQ ID NO: 149 - protein, 18 aa, Artificial Sequence
  GPC3B-110 HCDR3
ARYYWRGGSGQGSVTSDY

SEQ ID NO: 150 - protein, 7 aa, Artificial Sequence
  GPC3B-113 HCDR3
ARYSGDY

SEQ ID NO: 151 - protein, 13 aa, Artificial Sequence
  GPC3B-115 HCDR3
ARISGYHSSGWDY

SEQ ID NO: 152 - protein, 10 aa, Artificial Sequence
  GPC3B-119 HCDR3
ARGYYGKYDK

SEQ ID NO: 153 - protein, 7 aa, Artificial Sequence
  GPC3B-125 HCDR3
ARQSHDE

SEQ ID NO: 154 - protein, 8 aa, Artificial Sequence
  GPC3A-034 LCDR1
SSNIGSNN

SEQ ID NO: 155 - protein, 8 aa, Artificial Sequence
  GPC3A-035 LCDR1
SSNIGSNY

SEQ ID NO: 156 - protein, 8 aa, Artificial Sequence
  GPC3A-037 LCDR1
RSNIGSDY

SEQ ID NO: 157 - protein, 6 aa, Artificial Sequence
  GPC3A-038 LCDR1
NIGSKS

SEQ ID NO: 158 - protein, 6 aa, Artificial Sequence
  GPC3A-039 LCDR1
NIGSKS

SEQ ID NO: 159 - protein, 8 aa, Artificial Sequence
  GPC3A-040 LCDR1
SSNIGSNY

SEQ ID NO: 160 - protein, 8 aa, Artificial Sequence
  GPC3A-041 LCDR1
SSNIGSNY

SEQ ID NO: 161 - protein, 8 aa, Artificial Sequence
  GPC3A-042 LCDR1
SSDIGSNS

SEQ ID NO: 162 - protein, 8 aa, Artificial Sequence
  GPC3A-043 LCDR1
SSNIGTNY

SEQ ID NO: 163 - protein, 6 aa, Artificial Sequence
  GPC3A-044 LCDR1
NIGYKG

SEQ ID NO: 164 - protein, 8 aa, Artificial Sequence
  GPC3A-045 LCDR1
TSNIGTNT

SEQ ID NO: 165 - protein, 8 aa, Artificial Sequence
  GPC3A-046 LCDR1
SSNFGSNT

SEQ ID NO: 166 - protein, 8 aa, Artificial Sequence
  GPC3A-047 LCDR1
RSNIASND

SEQ ID NO: 167 - protein, 6 aa, Artificial Sequence
  GPC3A-048 LCDR1
NIGSKS

SEQ ID NO: 168 - protein, 8 aa, Artificial Sequence
  GPC3A-049 LCDR1
SSNIGSNY

SEQ ID NO: 169 - protein, 8 aa, Artificial Sequence
  GPC3A-050 LCDR1
SSNIGSNT

SEQ ID NO: 170 - protein, 9 aa, Artificial Sequence
  GPC3A-051 LCDR1
SSNIGAGYD

SEQ ID NO: 171 - protein, 8 aa, Artificial Sequence
  GPC3A-052 LCDR1
SSNIGSNY

SEQ ID NO: 172 - protein, 8 aa, Artificial Sequence
  GPC3A-053 LCDR1
SSNIGSNY

SEQ ID NO: 173 - protein, 8 aa, Artificial Sequence
  GPC3A-054 LCDR1
SSNIGSNY

SEQ ID NO: 174 - protein, 6 aa, Artificial Sequence
  GPC3A-055 LCDR1
NIGSKS

SEQ ID NO: 175 - protein, 6 aa, Artificial Sequence
  GPC3A-056 LCDR1
QSISSY

SEQ ID NO: 176 - protein, 6 aa, Artificial Sequence
  GPC3A-057 LCDR1
NIGSKS

SEQ ID NO: 177 - protein, 6 aa, Artificial Sequence
  GPC3A-058 LCDR1
NIGSKS

SEQ ID NO: 178 - protein, 6 aa, Artificial Sequence
  GPC3A-059 LCDR1
NIGSKS

SEQ ID NO: 179 - protein, 6 aa, Artificial Sequence
  GPC3A-060 LCDR1
NIGSES

SEQ ID NO: 180 - protein, 6 aa, Artificial Sequence
  GPC3A-061 LCDR1
NIGSKS

SEQ ID NO: 181 - protein, 9 aa, Artificial Sequence
  GPC3A-062 LCDR1
SSNIGAGYD

SEQ ID NO: 182 - protein, 8 aa, Artificial Sequence
  GPC3A-063 LCDR1
WSNIGSYT

SEQ ID NO: 183 - protein, 6 aa, Artificial Sequence
  GPC3A-064 LCDR1
NIGSKS

SEQ ID NO: 184 - protein, 6 aa, Artificial Sequence
  GPC3A-067 LCDR1
NIGSKS

SEQ ID NO: 185 - protein, 8 aa, Artificial Sequence
  GPC3B-54 LCDR1
NSNIGSDT

SEQ ID NO: 186 - protein, 6 aa, Artificial Sequence
  GPC3B-60 LCDR1
NLENKF

SEQ ID NO: 187 - protein, 11 aa, Artificial Sequence
  GPC3B-63 LCDR1
QSLLHSNGYNY

SEQ ID NO: 188 - protein, 6 aa, Artificial Sequence
  GPC3B-66 LCDR1
NIGSKS

SEQ ID NO: 189 - protein, 8 aa, Artificial Sequence
  GPC3B-68 LCDR1
SSNIGNNY

SEQ ID NO: 190 - protein, 6 aa, Artificial Sequence
  GPC3B-71 LCDR1
NIGSKS

SEQ ID NO: 191 - protein, 8 aa, Artificial Sequence
  GPC3B-76 LCDR1
SSNIGNNY

SEQ ID NO: 192 - protein, 6 aa, Artificial Sequence
  GPC3B-78 LCDR1
KLGDKY

SEQ ID NO: 193 - protein, 8 aa, Artificial Sequence
  GPC3B-80 LCDR1
SSNIGSNT

SEQ ID NO: 194 - protein, 6 aa, Artificial Sequence
  GPC3B-81 LCDR1
NIGSKS

SEQ ID NO: 195 - protein, 9 aa, Artificial Sequence
  GPC3B-82 LCDR1
SSNIGAGFD

SEQ ID NO: 196 - protein, 8 aa, Artificial Sequence
  GPC3B-85 LCDR1
SSNIGSNT

SEQ ID NO: 197 - protein, 11 aa, Artificial Sequence
  GPC3B-87 LCDR1
QSLLHSNGYNY

SEQ ID NO: 198 - protein, 6 aa, Artificial Sequence
  GPC3B-92 LCDR1
TLAKRY

SEQ ID NO: 199 - protein, 8 aa, Artificial Sequence
  GPC3B-93 LCDR1
SGSIASNY

SEQ ID NO: 200 - protein, 8 aa, Artificial Sequence
  GPC3B-110 LCDR1
SSNIGSNT

SEQ ID NO: 201 - protein, 8 aa, Artificial Sequence
  GPC3B-113 LCDR1
SSNIGSNS

SEQ ID NO: 202 - protein, 6 aa, Artificial Sequence
  GPC3B-115 LCDR1
NIGSKS

SEQ ID NO: 203 - protein, 8 aa, Artificial Sequence
  GPC3B-119 LCDR1
SSNIGNNY

SEQ ID NO: 204 - protein, 9 aa, Artificial Sequence
  GPC3B-125 LCDR1
SSDVGGYNY

SEQ ID NO: 205 - protein, 3 aa, Artificial Sequence
  GPC3A-034 LCDR2
SNH

SEQ ID NO: 206 - protein, 3 aa, Artificial Sequence
  GPC3A-035 LCDR2
KNF

SEQ ID NO: 207 - protein, 3 aa, Artificial Sequence
  GPC3A-037 LCDR2
GDN

SEQ ID NO: 208 - protein, 3 aa, Artificial Sequence
  GPC3A-038 LCDR2
YDS

SEQ ID NO: 209 - protein, 3 aa, Artificial Sequence
  GPC3A-039 LCDR2
YDS

SEQ ID NO: 210 - protein, 3 aa, Artificial Sequence
  GPC3A-040 LCDR2
SNN

SEQ ID NO: 211 - protein, 3 aa, Artificial Sequence
  GPC3A-041 LCDR2
KNF

SEQ ID NO: 212 - protein, 3 aa, Artificial Sequence
  GPC3A-042 LCDR2
STQ

SEQ ID NO: 213 - protein, 3 aa, Artificial Sequence
  GPC3A-043 LCDR2
RNN

SEQ ID NO: 214 - protein, 3 aa, Artificial Sequence
  GPC3A-044 LCDR2
DDS

SEQ ID NO: 215 - protein, 3 aa, Artificial Sequence
  GPC3A-045 LCDR2
SNN

SEQ ID NO: 216 - protein, 3 aa, Artificial Sequence
  GPC3A-046 LCDR2
SNT

SEQ ID NO: 217 - protein, 3 aa, Artificial Sequence
  GPC3A-047 LCDR2
KKN

SEQ ID NO: 218 - protein, 3 aa, Artificial Sequence
  GPC3A-048 LCDR2
YDS

SEQ ID NO: 219 - protein, 3 aa, Artificial Sequence
  GPC3A-049 LCDR2
RNN

SEQ ID NO: 220 - protein, 3 aa, Artificial Sequence
  GPC3A-050 LCDR2
SNN

SEQ ID NO: 221 - protein, 3 aa, Artificial Sequence
  GPC3A-051 LCDR2
GNS

SEQ ID NO: 222 - protein, 3 aa, Artificial Sequence
  GPC3A-052 LCDR2
RNN

SEQ ID NO: 223 - protein, 3 aa, Artificial Sequence
  GPC3A-053 LCDR2
GNS

SEQ ID NO: 224 - protein, 3 aa, Artificial Sequence
  GPC3A-054 LCDR2
RNN

SEQ ID NO: 225 - protein, 3 aa, Artificial Sequence
  GPC3A-055 LCDR2
YDS

SEQ ID NO: 226 - protein, 3 aa, Artificial Sequence
  GPC3A-056 LCDR2
AAS

SEQ ID NO: 227 - protein, 3 aa, Artificial Sequence
  GPC3A-057 LCDR2
YDS

SEQ ID NO: 228 - protein, 3 aa, Artificial Sequence
  GPC3A-058 LCDR2
DDS

SEQ ID NO: 229 - protein, 3 aa, Artificial Sequence
  GPC3A-059 LCDR2
YDS

SEQ ID NO: 230 - protein, 3 aa, Artificial Sequence
  GPC3A-060 LCDR2
DDD

SEQ ID NO: 231 - protein, 3 aa, Artificial Sequence
  GPC3A-061 LCDR2
YDS

SEQ ID NO: 232 - protein, 3 aa, Artificial Sequence
  GPC3A-062 LCDR2
GNS

SEQ ID NO: 233 - protein, 3 aa, Artificial Sequence
  GPC3A-063 LCDR2
GNN

SEQ ID NO: 234 - protein, 3 aa, Artificial Sequence
  GPC3A-064 LCDR2
DDT

SEQ ID NO: 235 - protein, 3 aa, Artificial Sequence
  GPC3A-067 LCDR2
YDS

SEQ ID NO: 236 - protein, 3 aa, Artificial Sequence
  GPC3B-54 LCDR2
RDN

SEQ ID NO: 237 - protein, 3 aa, Artificial Sequence
  GPC3B-60 LCDR2
EDN

SEQ ID NO: 238 - protein, 3 aa, Artificial Sequence
  GPC3B-63 LCDR2
LGS

SEQ ID NO: 239 - protein, 3 aa, Artificial Sequence
  GPC3B-66 LCDR2
YDS

SEQ ID NO: 240 - protein, 3 aa, Artificial Sequence
  GPC3B-68 LCDR2
DNI

SEQ ID NO: 241 - protein, 3 aa, Artificial Sequence
  GPC3B-71 LCDR2
YDS

SEQ ID NO: 242 - protein, 3 aa, Artificial Sequence
  GPC3B-76 LCDR2
DNN

SEQ ID NO: 243 - protein, 3 aa, Artificial Sequence
  GPC3B-78 LCDR2
QDN

SEQ ID NO: 244 - protein, 3 aa, Artificial Sequence
  GPC3B-80 LCDR2
SNN

SEQ ID NO: 245 - protein, 3 aa, Artificial Sequence
  GPC3B-81 LCDR2
YDS

SEQ ID NO: 246 - protein, 3 aa, Artificial Sequence
  GPC3B-82 LCDR2
DNN

SEQ ID NO: 247 - protein, 3 aa, Artificial Sequence
  GPC3B-85 LCDR2
SNN

SEQ ID NO: 248 - protein, 3 aa, Artificial Sequence
  GPC3B-87 LCDR2
LGS

SEQ ID NO: 249 - protein, 3 aa, Artificial Sequence
  GPC3B-92 LCDR2
RDT

SEQ ID NO: 250 - protein, 3 aa, Artificial Sequence
  GPC3B-93 LCDR2
EDN

SEQ ID NO: 251 - protein, 3 aa, Artificial Sequence
  GPC3B-110 LCDR2
SSN

SEQ ID NO: 252 - protein, 3 aa, Artificial Sequence
  GPC3B-113 LCDR2
SNN

SEQ ID NO: 253 - protein, 3 aa, Artificial Sequence
  GPC3B-115 LCDR2
DDS

SEQ ID NO: 254 - protein, 3 aa, Artificial Sequence
  GPC3B-119 LCDR2
DNN

SEQ ID NO: 255 - protein, 3 aa, Artificial Sequence
  GPC3B-125 LCDR2
EVS

SEQ ID NO: 256 - protein, 11 aa, Artificial Sequence
  GPC3A-034 LCDR3
AAWDDSLDGYL

SEQ ID NO: 257 - protein, 11 aa, Artificial Sequence
  GPC3A-035 LCDR3
AAWDDALSGYV

SEQ ID NO: 258 - protein, 11 aa, Artificial Sequence
  GPC3A-037 LCDR3
GTWDYTLNGVV

SEQ ID NO: 259 - protein, 11 aa, Artificial Sequence
  GPC3A-038 LCDR3
QVWDSSSDHVV

SEQ ID NO: 260 - protein, 11 aa, Artificial Sequence
  GPC3A-039 LCDR3
QVWDSSSDHWV

SEQ ID NO: 261 - protein, 11 aa, Artificial Sequence
  GPC3A-040 LCDR3
AAWDDSLSGYV

SEQ ID NO: 262 - protein, 11 aa, Artificial Sequence
  GPC3A-041 LCDR3
AAWDDALSGYV

SEQ ID NO: 263 - protein, 11 aa, Artificial Sequence
  GPC3A-042 LCDR3
ATWDDSLNGYV

SEQ ID NO: 264 - protein, 11 aa, Artificial Sequence
  GPC3A-043 LCDR3
AVWDDSLSGVV

SEQ ID NO: 265 - protein, 11 aa, Artificial Sequence
  GPC3A-044 LCDR3
QVWDSSSDHVV

SEQ ID NO: 266 - protein, 11 aa, Artificial Sequence
  GPC3A-045 LCDR3
AAWDDSLNGVV

SEQ ID NO: 267 - protein, 11 aa, Artificial Sequence
  GPC3A-046 LCDR3
AAWDDSLTGVV

SEQ ID NO: 268 - protein, 11 aa, Artificial Sequence
  GPC3A-047 LCDR3
AAWDDNLSGYV

SEQ ID NO: 269 - protein, 11 aa, Artificial Sequence
  GPC3A-048 LCDR3
QVWDSSSDRGV

SEQ ID NO: 270 - protein, 9 aa, Artificial Sequence
  GPC3A-049 LCDR3
AAWDDSLSG

SEQ ID NO: 271 - protein, 11 aa, Artificial Sequence
  GPC3A-050 LCDR3
AAWDDSLNGPV

SEQ ID NO: 272 - protein, 11 aa, Artificial Sequence
  GPC3A-051 LCDR3
QSYDSSLSGYV

SEQ ID NO: 273 - protein, 11 aa, Artificial Sequence
  GPC3A-052 LCDR3
AAWDDSLSGYV

SEQ ID NO: 274 - protein, 12 aa, Artificial Sequence
  GPC3A-053 LCDR3
QSYDSSLSGSNV

SEQ ID NO: 275 - protein, 11 aa, Artificial Sequence
  GPC3A-054 LCDR3
AAWDDSLSGYV

SEQ ID NO: 276 - protein, 11 aa, Artificial Sequence
  GPC3A-055 LCDR3
QVWDSSSDHYV

SEQ ID NO: 277 - protein, 9 aa, Artificial Sequence
  GPC3A-056 LCDR3
QQSYSTPIT

SEQ ID NO: 278 - protein, 11 aa, Artificial Sequence
  GPC3A-057 LCDR3
QVWDSSSDHVV

SEQ ID NO: 279 - protein, 10 aa, Artificial Sequence
  GPC3A-058 LCDR3
QVWDSSSDHV

SEQ ID NO: 280 - protein, 10 aa, Artificial Sequence
  GPC3A-059 LCDR3
QVWDSSSDHV

SEQ ID NO: 281 - protein, 9 aa, Artificial Sequence
  GPC3A-060 LCDR3
QTWDSSTAI

SEQ ID NO: 282 - protein, 11 aa, Artificial Sequence
  GPC3A-061 LCDR3
QVWDSSSDHYV

SEQ ID NO: 283 - protein, 12 aa, Artificial Sequence
  GPC3A-062 LCDR3
QSYDSSLSGSYV

SEQ ID NO: 284 - protein, 11 aa, Artificial Sequence
  GPC3A-063 LCDR3
AAWDDNLNGVV

SEQ ID NO: 285 - protein, 11 aa, Artificial Sequence
  GPC3A-064 LCDR3
QVWDRSSAHWV

SEQ ID NO: 286 - protein, 11 aa, Artificial Sequence
  GPC3A-067 LCDR3
QVWDSSSDHVV

SEQ ID NO: 287 - protein, 11 aa, Artificial Sequence
  GPC3B-54 LCDR3
TTWDDSLNGLV

SEQ ID NO: 288 - protein, 11 aa, Artificial Sequence
  GPC3B-60 LCDR3
QTWDSPTGLFV

SEQ ID NO: 289 - protein, 9 aa, Artificial Sequence
  GPC3B-63 LCDR3
MQALQTPPT

SEQ ID NO: 290 - protein, 12 aa, Artificial Sequence
  GPC3B-66 LCDR3
QVWDSSSDHLYV

SEQ ID NO: 291 - protein, 11 aa, Artificial Sequence
  GPC3B-68 LCDR3
GTWDSSLSAGV

SEQ ID NO: 292 - protein, 11 aa, Artificial Sequence
  GPC3B-71 LCDR3
QVWDSSSDHYV

SEQ ID NO: 293 - protein, 11 aa, Artificial Sequence
  GPC3B-76 LCDR3
GTWDSSLSAGV

SEQ ID NO: 294 - protein, 9 aa, Artificial Sequence
  GPC3B-78 LCDR3
QTWDRSTYV

SEQ ID NO: 295 - protein, 9 aa, Artificial Sequence
  GPC3B-80 LCDR3
AAWDDSLNG

SEQ ID NO: 296 - protein, 12 aa, Artificial Sequence
  GPC3B-81 LCDR3
QVWDSSSDLLYV

SEQ ID NO: 297 - protein, 11 aa, Artificial Sequence
  GPC3B-82 LCDR3
QSFDSSLSGWV

SEQ ID NO: 298 - protein, 11 aa, Artificial Sequence
  GPC3B-85 LCDR3
AAWDDSLNGYV

SEQ ID NO: 299 - protein, 9 aa, Artificial Sequence
  GPC3B-87 LCDR3
MQALQTPWT

SEQ ID NO: 300 - protein, 10 aa, Artificial Sequence
  GPC3B-92 LCDR3
QSADNSRTFV

SEQ ID NO: 301 - protein, 9 aa, Artificial Sequence
  GPC3B-93 LCDR3
QSYDSSNWV

SEQ ID NO: 302 - protein, 11 aa, Artificial Sequence
  GPC3B-110 LCDR3
AAWDDSLNGPV

SEQ ID NO: 303 - protein, 11 aa, Artificial Sequence
  GPC3B-113 LCDR3
AAWDDSLNGVL

SEQ ID NO: 304 - protein, 12 aa, Artificial Sequence
  GPC3B-115 LCDR3
QVWDSSSDPLYV

SEQ ID NO: 305 - protein, 11 aa, Artificial Sequence
  GPC3B-119 LCDR3
ATWDNSLSALI

SEQ ID NO: 306 - protein, 10 aa, Artificial Sequence
  GPC3B-125 LCDR3
SSYTSSTTVI

SEQ ID NO: 307 - protein, 116 aa, Artificial Sequence
  GPC3A-034 VH
QVQLQQWGAGLLKPSETLSLTCAVYGGSFSGYYWSWIRQPPGKGLEWIGEINHSGSTNYNPSLKSRVTISVDTSKNQFSLELSSVTAADTAVYYCARGYGGRFDYWGQGTLVTVSS

SEQ ID NO: 308 - protein, 117 aa, Artificial Sequence
  GPC3A-035 VH
QVQLVQSGAEVKKPGASVKVSCKASGYTFTGYYMHWVRQAPGQGLEWMGWINPNSGGTNYAQKFQGRVTMTRDTSISTAYMELSRLRSDDTAVYYCARSWTSGFDYWGQGTLVTVSS

SEQ ID NO: 309 - protein, 118 aa, Artificial Sequence
  GPC3A-037 VH
QVQLVESGGGLVQPGGSLRLSCAASGFTFSSYAMSWVRQAPGKGLEWVSVIYSGGSSTYYADSVKGRFTISRDNSKNTLYLQMNSLRAEDTAVYYCARTSYLNHGDYWGQGTLVTVSS

SEQ ID NO: 310 - protein, 116 aa, Artificial Sequence
  GPC3A-038 VH
QVQLVQSGAEVKKPGASVKVSCKASGYTFTSYYMHWVRQAPGQGLEWMGIINPSGGSTSYAQKFQGRVTMTRDTSTSTVYMELSSLRSEDTAVYYCARKVTGYDSWGQGTLVTVSS

SEQ ID NO: 311 - protein, 116 aa, Artificial Sequence
  GPC3A-039 VH
QVQLVQSGGGLVHPGGSLRLSCAGSGFTFSSYAMHWVRQAPGKGLEWVSAIGTGGGTYYADSVKGRFTISRDNAKNSLYLQMNSLRAEDTAVYYCARYGRKSIDAWGQGTLVTVSS

SEQ ID NO: 312 - protein, 117 aa, Artificial Sequence
  GPC3A-040 VH
QVQLVQSGAEVKKPGASVTVSCKASGYTFTGYYMHWVRQAPGQGLEWMGWINPNSGGTNYAQKFQGRVTMTRDTSISTAYMELSRLRSDDTAVYYCARRGYYGYDSWGQGTLVTVSS

SEQ ID NO: 313 - protein, 117 aa, Artificial Sequence
  GPC3A-041 VH
EVQLVQSGAEVKKPGASVKVSCKASGYTFTGYYMHWVRQAPGQGLEWMGWINPNSGGTNYAQKFQGRVTMTRDTSISTAYMELSRLRSDDTAMYYCARSGKYYGDKWGQGTLVTVSS

SEQ ID NO: 314 - protein, 117 aa, Artificial Sequence
  GPC3A-042 VH
QVQLQQSGAEVKKPGASVKVSCKASGYSFTGYYVYWMRQAPGKGLEWMGWMNPRSGGTNYAQKFQGRVTMTRDTSISTAYMELSRLTSDDTAVYYCARSSYYWADSWGQGTLVTVSS

SEQ ID NO: 315 - protein, 124 aa, Artificial Sequence
  GPC3A-043 VH
EVQLVQSGAEVKKPGATVKVSCKVSGYTFTDYYMHWVQQAPGKGLEWMGLVDPEDGETIYAEKFQGRVTITADTSTDTAYMELSSLRSEDTAVYYCARELRDVAYYPWGVEDFWGQGTLVTVSS

SEQ ID NO: 316 - protein, 116 aa, Artificial Sequence
  GPC3A-044 VH
QVQLQQWGAGLLKPSETLSLTCAVYGGSFSGYYWSWIRQPPGKGLEWIGEINHSGSTNYNPSLKSRVTISVDTSKNQFSLKLSSVTAADTAVYYCARYYVPYLSDWGQGTLVTVSS

SEQ ID NO: 317 - protein, 116 aa, Artificial Sequence
  GPC3A-045 VH
QMQLVQSGGGLVKPGGSLRLSCAASGFTFSDYYMSWIRQAPGKGLEWVSYISSSGSTIYYADSVKGRFTISRDNAKNSLYLQMNSLRAEDTAVYYCARASDLYGDWGQGTLVTVSS

SEQ ID NO: 318 - protein, 121 aa, Artificial Sequence
  GPC3A-046 VH
QVQLVQSGAEVKKPGASVTVSCKASGYRFSNYGVSWVRQAPGQGLEWMGWISGSNGNTNYAQKFLGRVTMTTDTSTTTAYMELSSLRSDDTAVYYCARGNRRYYSPIIDPWGQGTLVTVSS

SEQ ID NO: 319 - protein, 118 aa, Artificial Sequence
  GPC3A-047 VH
QVQLVQSGAEVKKPGASVKVSCKAPGYTFTGYYMHWVRQAPGQGLEWMGWINPNSGGTNYAQKFQGRVTMTRDTSISTAYMELSRLRSDDTAVYYCARSDYGSLYDKWGQGTLVTVSS

SEQ ID NO: 320 - protein, 117 aa, Artificial Sequence
  GPC3A-048 VH
EVQLVESGGGEVQPGRSLRLSCAASGFTFSSYAMHWVRQAPGKGLEWVAVISYDGSNKYYADSVKGRFTISRDNSKNTLYLQMNSLRAEDTAVYYCARSSFVATDYWGQGTLVTVSS

SEQ ID NO: 321 - protein, 121 aa, Artificial Sequence
  GPC3A-049 VH
QVQLVQSGAEVKEPGASVKVSCKASGYTFTGYYMHWVRQAPGQGLEWMGWINPNSGGTNYAQKFQGRVTMTRDTSISTAYMELSRLRSDDTAVYYCARHGGIGSMRSFDQWGQGTLVTVSS

SEQ ID NO: 322 - protein, 117 aa, Artificial Sequence
  GPC3A-050 VH
QITLKESGAEVKKPGASVKVSCKASGYSFTGYYVYWMRQAPGKGLEWMGWMNPRSGGTNYAQKFQGRVTMTRDTSISTAYMELSRLTSDDTATYYCARSGYRWLDVWGQGTLVTVSS

SEQ ID NO: 323 - protein, 121 aa, Artificial Sequence
  GPC3A-051 VH
QVQLVQSGAEVKKPGSSVKVSCKASGGAFSSYAISWVRQAPGQGLEWMGGIIPIFGTANYAQKFQGRVTITADESTSTAYMELSSLRSEDTAVYYCARMLYLSGRYYWDSWGQGTLVTVSS

SEQ ID NO: 324 - protein, 117 aa, Artificial Sequence
  GPC3A-052 VH
EVQLVESGAEVKKPGASVKVSCKASGYTFTGYYMHWVRQAPGQGLEWMGWINPNSGGTNYAQKFQGRVTMTRDTSISTAYMELSRLRSDDTAVYYCARSHSSGYDKWGQGTLVTVSS

SEQ ID NO: 325 - protein, 118 aa, Artificial Sequence
  GPC3A-053 VH
QLQLQESGPGLVKPSETLSLTCTVSGGSISSSSYYWGWIRQPPGKGLEWIGSIYYSGSTYYNPSLKSRVTISVDTSKNQFSLKLSSVTAADTAVYYCARWWSGSYDTWGQGTLVTVSS

SEQ ID NO: 326 - protein, 119 aa, Artificial Sequence
  GPC3A-054 VH
QMQLVQSGAEVKKPGASVKVSCKASGYTFTSYGISWVRQAPGQGLEWMGWISAYNGNTNYAQKLQGRVTMTTDTSTSTAYMELRSLRSDDTAVYYCARIPMYSGSSDYWGQGTLVTVSS

SEQ ID NO: 327 - protein, 117 aa, Artificial Sequence
  GPC3A-055 VH
QVQLVQSGAEVKKPGASVKVSCKASGYTFTSYYMHWVRQAPGQGLEWMGIINPSGGSTSYAQKFQGRVTMTRDTSTSTVYMELSSLRSEDTAVYYCARWHGGPYDYWGQGTLVTVSS

SEQ ID NO: 328 - protein, 122 aa, Artificial Sequence
  GPC3A-056 VH
QVQLQQSGAEVKKFGASVKVSCKASGYSFNDYYIHWVRQAPGQGLEWMGWINPNNGDTKYEKKWQGRVTMTRDTSITTAYMELSSLRSDDTAVYYCARFSTHNWWWPTYDYWGQGTLVTVSS

SEQ ID NO: 329 - protein, 120 aa, Artificial Sequence
  GPC3A-057 VH
EVQLVESGGGLIQPGGSLRLSCAASGFTFSSYAMSWVRQAPGKGLEWVSAISGSGGSTYYADSVKGRFTISRDNSKNTLYLQMNSLRAEDTAVYYCARYNYMSSGFYDRWGQGTLVTVSS

SEQ ID NO: 330 - protein, 120 aa, Artificial Sequence
  GPC3A-058 VH
QVQLVQSGADVRKPGASVKVSCKASGYTFASHGISWVRQAPGQGLEWLGWISPYTGNTNYAQKFQGRVTMATDTSTSTAYMELRSLRSDDTAIYYCARGKRTLASCFDYWGQGTLVTVSS

SEQ ID NO: 331 - protein, 117 aa, Artificial Sequence
  GPC3A-059 VH
QVQLVQSGAEVKKPGASVTVSCKASGYTFTRYGITWVRQAPGQGLEWMGWISAYSDKTNYAQKLQGRVTMTTDISTNTAYMELSSLRSEDTAVYYCARSRWSYMDVWGQGTLVTVSS

SEQ ID NO: 332 - protein, 119 aa, Artificial Sequence
  GPC3A-060 VH
QVQLVQSGGEVKKPGASVKVSCKASGYTFNSYAISWVRQAPGQGLEWMGWISAYNGNTNYAQKLQGRVTMTTDTSTNTAFMELRSLRSDDTAVYYCAREGYGSWAMDQWGQGTLVTVSS

SEQ ID NO: 333 - protein, 117 aa, Artificial Sequence
  GPC3A-061 VH
QVQLVQSGAEVKKPGASVKVSCKASGYTFTSYGISWVRQTPGQGLEWMGWISAYNGNTNYAQKLQGRVTMTTDTSTSTAYMELSSLRSEDTAVYYCARKGSSQFDQWGQGTLVTVSS

SEQ ID NO: 334 - protein, 123 aa, Artificial Sequence
  GPC3A-062 VH
QMQLVQSGSELKKPGASVKVSCKASGGTFSSYAISWVRQAPGQGLEWMGGIIPKIGTANYAQKFQGRVTITADESTSTAYMELSSLRSEDTAMYYCARMYMDMGWGWGYWDWWGQGTLVTVSS

SEQ ID NO: 335 - protein, 119 aa, Artificial Sequence
  GPC3A-063 VH
QVQLVQSGAEVKKPGASVKVSCKASGYTFTSYYMHWVRQAPGQGLEWMGIINPSGGSASYAQKFQGRVTMTRDTSTSTVYMELSSLRSEDTAVYYCARDRLASDAFDIWGQGTMVTVSS

SEQ ID NO: 336 - protein, 120 aa, Artificial Sequence
  GPC3A-064 VH
QMQLVQSGAEVKKPGASVKVSCKASGYTFTIYGISWVRQAPGQGLEWMGWISPYNDNTIYAQKVQGRVTMTTDTSTSTAYMELRSLRSDDTAVYYCARMGVGWGYAQDSWGQGTLVTVSS

SEQ ID NO: 337 - protein, 116 aa, Artificial Sequence
  GPC3A-067 VH
EVQLVQSGAEVKKPGSSVKVSCKASGGTFSSYAISWVRQAPGQGLEWMGRIIPIFGITNYAQKFQGRVTITADKSTSTAYMELSSLRSEDTAVYYCARGAEMSDYWGQGTLVTVSS

SEQ ID NO: 338 - protein, 120 aa, Artificial Sequence
  GPC3B-54 VH
EVQLVQSGAEVKKPGASVKLSCKTSGYTFIDYYVYWVRQAPGQGLEWMGGIIPIFGTANYAQKFQGRVTITADKSTSTAYMELSSLGSEDTAVYYCARERRYSSSPSDHWGQGTLVTVSS

SEQ ID NO: 339 - protein, 119 aa, Artificial Sequence
  GPC3B-60 VH
EVQLVESGAEVKKPGASVKVSCKASGYTFTSYYMHWVRQAPGQGLEWMGIINPSGGSTSYAQKFQGRVTMTRDTSTSTVYMELSSLRSEDTAVYYCARSLYSQPYIDGWSQGTLVTVSS

SEQ ID NO: 340 - protein, 122 aa, Artificial Sequence
  GPC3B-63 VH
QVQLVQSGAEVKKPGASVKVSCKASGYTFTSYYMHWVRQAPGQGLEWMGIINPSGGSTSYAQKFQGRVTMTRDTSTSTVYMELSSLRSEDTAVYYCARSLHAMRWSQTMDSWGQGTLVTVSS

SEQ ID NO: 341 - protein, 118 aa, Artificial Sequence
  GPC3B-66 VH
QVQLVQSGAEVKRPGASVKVSCKASGYTFIGQYLHWVRQAPGQGLEWMGRINPMTGVTNYAPKFQGRVTMTRDTSISTGYMEISRLRSDDTAVYYCARFSSGYSRDTWGQGTLVTVSS

SEQ ID NO: 342 - protein, 117 aa, Artificial Sequence
  GPC3B-68 VH
QVQLVQSGAEVKKPGSSVKVSCKASGGTFSSYAISWVRQAPGQGLEWMGRIIPILGIANYAQKFQGRVTITADKSTSTAYMELSSLRSEDTAVYYCARYGYEGHDTWGQGTLVTVSS

SEQ ID NO: 343 - protein, 120 aa, Artificial Sequence
  GPC3B-71 VH
EVQLVESGGGLVKPGGSLRLSCAASGFTFSRYTMNWVRQAPGKGLEWVSSISSSGSYIYYADSVKGRFTISRDNAKNSLFLQMDSLRAEDTAVYYCARQGHMWYVPVDAWGQGTLVTVSS

SEQ ID NO: 344 - protein, 112 aa, Artificial Sequence
  GPC3B-76 VH
QMQLVQSGAEVKEPGASVKVSCKASGYTFTDYYIHWVRQAPGQGLEWMGWINPNSGGTNYAQKFQGRVTMTRDTSISTAYMELSRLRSDDTAVYYCARNYDWGQGTLVTVSS

SEQ ID NO: 345 - protein, 117 aa, Artificial Sequence
  GPC3B-78 VH
QMQLVQSGAEVKKPGASVKVSCKASGYTFTSYYMHWVRQAPGQGLEWMGIINPSGGSTSYAQKFQGRVTMTRDTSTSTVYMELSSLRSEDTAVYYCARGYSSFFDSWGQGTLVTVSS

SEQ ID NO: 346 - protein, 122 aa, Artificial Sequence
  GPC3B-80 VH
QVQLVQSGAEVKKPGSSVKVSCKASGGTLSRFAISWVRQAPGQGLEWMGGIIPIFRTANYAQKFQGRVTITADESTSTAYMELSSLRSEDTAVYYCARMSKYYGSYSSYDEWGQGTLVTVSS

SEQ ID NO: 347 - protein, 114 aa, Artificial Sequence
  GPC3B-81 VH
EVQLVQSGAEVKKPGASVKVSCKASGYTFTGYYMHWVRQAPGQGLEWMGRINPNSGGTNYAQKFQGRVTMTRDTSISTAYMELSRLRSDDTAVYYCARGLWDSWGQGTLVTVSS

SEQ ID NO: 348 - protein, 121 aa, Artificial Sequence
  GPC3B-82 VH
EVQLVQSGAEVKKPGESLKISCKGSGYSFTSYYMHWVRQAPGQGLEWMGIINPSGGSTSYAQKFQGRVTMTRDTSTSTVYMEMSSLRSEDTAVYYCARYPVYMETSDFDSWGSRYSGDRLL

SEQ ID NO: 349 - protein, 125 aa, Artificial Sequence
  GPC3B-85 VH
QVQLVQSGSELKKPGASVKVSCKASGYTFTSYAMNWVRQAPGQGLEWMGWINTNTGNPTYAQGFTGRFVFSLDTSVSTAYLQISSLKAEDTAVYYCARSSLYWMGSKWSRQTDMWGQGTLVTVSS

SEQ ID NO: 350 - protein, 113 aa, Artificial Sequence
  GPC3B-87 VH
EVQLVQSGAEVRKPGSSVKVSCQASGGTFGSYAISWVRQAPGQGLEWMGRIIPVLGRTKYAQKFQGRVTVTADTSTSTVYMELTSLTSEDTAVYYCARTNDSWGQGTLVTVSS

SEQ ID NO: 351 - protein, 120 aa, Artificial Sequence
  GPC3B-92 VH
EVQLVQSGAEVKKPGASVKVSCKASGYTFSNYYMHWVRQAPGQGLEWMGIINPSGGTTTYAQKFQGRVTMTRDTSTSTVYMELSSLRSEDTAVYYCARPSMWTSSMGDVWGQGTLVTVSS

SEQ ID NO: 352 - protein, 123 aa, Artificial Sequence
  GPC3B-93 VH
EVQLVQSGAEVKKPGASVKVSCKASGYTFTSYYMHWVRQAPGQGLEWMGIINPSGGSTRYAQKFQGRVTMTRDTSTSTVYMELSSLRSEDTAVYYCARYTALKPRGIYSVDSWGQGTLVTVSS

SEQ ID NO: 353 - protein, 125 aa, Artificial Sequence
  GPC3B-110 VH
EVQLVQSGAEVKKPGSSVKVSCQASGGTFTTYSINWVRQAPGQGLEWMGGIIPTFGTTNYAQNFQDRVTISADESTNTAYMELTSLRSEDTAVYYCARYYWRGGSGQGSVTSDYWGQGTLVTVSS

SEQ ID NO: 354 - protein, 114 aa, Artificial Sequence
  GPC3B-113 VH
QVQLVQSGAEVKKPGASVKVSCKVSGYTLTELSMHWVRQAPGKGLEWMGGFDPEDGETIYAQKFQGRVTMTEDTSTDTAYMELSSLRSEDTAVYYCARYSGDYWGQGTLVTVSS

SEQ ID NO: 355 - protein, 120 aa, Artificial Sequence
  GPC3B-115 VH
QVQLVQSGAEVKRPGATIKVSCKTSGYTFTAYYTHWVRQAPGQGLEWVGRINANTGGTDYAPKFRDRVIMTRDTSISTAYMELGRLTSEDTAVYYCARISGYHSSGWDYWGQGTLVTVSS

SEQ ID NO: 356 - protein, 117 aa, Artificial Sequence
  GPC3B-119 VH
QVQLVQSGSELKKPGASVKVSCKASGYTFTSYAMNWVRQAPGQGLEWMGWINTNTGNPTYAQGFTGRFVFSLDTSVSTAYLQISSLKAEDTAVYYCARGYYGKYDKWGQGTLVTVSS

SEQ ID NO: 357 - protein, 114 aa, Artificial Sequence
  GPC3B-125 VH
QMQLVQSGSELKKPGASVKVSCKASGYTFTSYAMNWVRQAPGQGLEWMGWINTNTGNPTYAQGFTGRFVFSLDTSVSTAYLQISSLKAEDTAVYYCARQSHDEWGQGTLVTVSS

SEQ ID NO: 358 - protein, 111 aa, Artificial Sequence
  GPC3A-034 VL
QPVLTQPPSASGTPGQRVTISCSGSSSNIGSNNVIWYQQLPGAAPKLLIYSNHRRPSGVPDRFSGSRSGTSASLAISGLQSEDEADYYCAAWDDSLDGYLFGTGTKVTVLG

SEQ ID NO: 359 - protein, 111 aa, Artificial Sequence
  GPC3A-035 VL
QAVLTQPPSASQTPGQMVTISCSGTSSNIGSNYVFWYQQLPGTAPKLLIYKNFQRPSGVPGRFSGSKSGTAASLAISGLRSEDEADYFCAAWDDALSGYVFGAGTKVTVLG

SEQ ID NO: 360 - protein, 111 aa, Artificial Sequence
  GPC3A-037 VL
QSVLTQPPSVSAAPGQRVTISCSGTRSNIGSDYVSWYQHLPGTAPKLLVYGDNLRPSGIPDRFSASKSGTSATLGITGLQTGDEADYYCGTWDYTLNGVVFGGGTKLTVLG

SEQ ID NO: 361 - protein, 109 aa, Artificial Sequence
  GPC3A-038 VL
QSVLTQPPSVSVAPGKTARITCGGNNIGSKSVHWYQQKPGQAPVLVIYYDSDRPSGIPERFSGSNSGNTATLTISRVEAGDEADYYCQVWDSSSDHVVFGGGTKLTVLG

SEQ ID NO: 362 - protein, 109 aa, Artificial Sequence
  GPC3A-039 VL
SYVLTQPPSVSVAPGKTARITCGGNNIGSKSVHWYQQKPGQAPVLVIYYDSDRPSGIPERFSGSNSGNTATLTISRVEAGDEADYYCQVWDSSSDHWVFGGGTKLTVLG

SEQ ID NO: 363 - protein, 111 aa, Artificial Sequence
  GPC3A-040 VL
LPVLTQPPSASGTPGQRVTISCSGSSSNIGSNYVYWYQQLPGTAPKLLIYSNNQRPSGVPDRFSGSKSGTSASLAISGLRSEDEADYYCAAWDDSLSGYVFGTGTKVTVLG

SEQ ID NO: 364 - protein, 111 aa, Artificial Sequence; identical to SEQ ID NO: 359
  GPC3A-041 VL

SEQ ID NO: 365 - protein, 111 aa, Artificial Sequence
  GPC3A-042 VL
SYVLTQPPSASGTPGQRVTISCFGSSSDIGSNSVFWYQQLPGAAPKLLIYSTQYRPSGVPDRFSGSKSGTSASLAISGLQSEDEAEYHCATWDDSLNGYVFGSGTKVTVLG

SEQ ID NO: 366 - protein, 111 aa, Artificial Sequence
  GPC3A-043 VL
QSVLTQPPSASGTPGQRVTISCSGSSSNIGTNYVYWYQQLPGTAPKLIIYRNNQRPSGVPDRFSGSESGTSASLAISGLRSEDEADYYCAVWDDSLSGVVFGGGTKLTVLG

SEQ ID NO: 367 - protein, 109 aa, Artificial Sequence
  GPC3A-044 VL
SYVLTQPPSVSVAPGKTARITCGGDNIGYKGVHWYQQKPGQAPVLVVYDDSDRPSGIPERFSGSNSGNTATLTISRVEAGDEADYYCQVWDSSSDHVVFGGGTKLTVLG

SEQ ID NO: 368 - protein, 111 aa, Artificial Sequence
  GPC3A-045 VL
QSVLTQPPSVSGTPGQRVIISCPGSTSNIGTNTVNWYQQFPGTAPKLLIYSNNQRPSGVPDRFSGSKSGTSASLAISGLQSEDEADYYCAAWDDSLNGVVFGGGTKLTVLG

SEQ ID NO: 369 - protein, 111 aa, Artificial Sequence
  GPC3A-046 VL
QAVLTQPPSVSGTPGQRVTISCSGSSSNFGSNTVHWYQQVPGTAPKLLIFSNTQRPSEIPDRFSGSKSGTSASLAISGLQSEDEADYYCAAWDDSLTGVVFGGGTKLTVLG

SEQ ID NO: 370 - protein, 111 aa, Artificial Sequence
  GPC3A-047 VL
LPVLTQPPSASGTPGQRVTISCSGSRSNIASNDVYWYQQLPGTAPKRLIYKKNQRPSGVPDRFSASKSGTSASLAISGLRSEDEADYYCAAWDDNLSGYVFGTGTKVTVLG

SEQ ID NO: 371 - protein, 109 aa, Artificial Sequence
  GPC3A-048 VL
QPVLTQPPSVSVAPGKTARITCGGNNIGSKSVHWYQQKPGQAPVLVIYYDSDRPSGIPERFSGSNSGNTATLTISRVEAGDEADFYCQVWDSSSDRGVFGGGTKLTVLG

SEQ ID NO: 372 - protein, 111 aa, Artificial Sequence
  GPC3A-049 VL
QAVLTQPSSASGTPGQRVTISCSGGSSNIGSNYVYWYQQLPGTAPKLLIYRNNQRPSGVPDRFSGSKSGTSASLAISGLRSEDEADYYCAAWDDSLSGWVFGGRTKLTVLG

SEQ ID NO: 373 - protein, 111 aa, Artificial Sequence
  GPC3A-050 VL
QAVLTQPSSASGTPGQRVTISCSGSSSNIGSNTVNWYQQLPGTAPKLLIYSNNQRPSGVPDRFSGSKSGTSASLAISGLQSEDEADYYCAAWDDSLNGPVFGTGTKVTVLG

SEQ ID NO: 374 - protein, 112 aa, Artificial Sequence
  GPC3A-051 VL
QAVLTQPSSASGAPGQRVTISCTGGSSNIGAGYDVHWYQQLPGTAPKLLIYGNSNRPSGVPDRFSGSKSGTSASLAITGLQAEDEADYYCQSYDSSLSGYVFGTGTKVTVLG

SEQ ID NO: 375 - protein, 111 aa, Artificial Sequence
  GPC3A-052 VL
QAVLTQPSSASGTPGQRVTISCSGSSSNIGSNYVYWYQQLSGTAPKLLIYRNNQRPSGVPDRFSGSKSGTSASLAISGLRSEDEADYYCAAWDDSLSGYVFGTGTKVTVLG

SEQ ID NO: 376 - protein, 112 aa, Artificial Sequence
  GPC3A-053 VL
QSVLTQPPSASAAPGQRVTISCSGTSSNIGSNYVWWYQQLPGAAPRLLIYGNSNRPSGVPDRFSGSKSGTSASLAITGLQAEDEADYYCQSYDSSLSGSNVFGTGTKVTVLG

SEQ ID NO: 377 - protein, 111 aa, Artificial Sequence
  GPC3A-054 VL
SYELTQPPSASGTPGQRVTISCSGSSSNIGSNYVYWYQQLPGTAPKLLIYRNNQRPSGVPDRFSGSKSGTSASLAISGLRSEDEADYYCAAWDDSLSGYVFGTGTKVTVLG

SEQ ID NO: 378 - protein, 109 aa, Artificial Sequence
  GPC3A-055 VL
QPVLTQPPSVSVAPGKTARITCGGNNIGSKSVHWYQQKPGQAPVLVIYYDSDRPSGIPERFSGSNSGNTATLTISRVEAGDEADYYCQVWDSSSDHYVFGTGTKVTVLG

SEQ ID NO: 379 - protein, 108 aa, Artificial Sequence
  GPC3A-056 VL
DIQLTQSPSSLSASVGDRVTITCRASQSISSYLNWYQQKPGKAPKLLIYAASSLQSGVPSRFSGSGSGTDFTLTISSLQPEDFATYYCQQSYSTPITFGQGTRLEIKR

SEQ ID NO: 380 - protein, 109 aa, Artificial Sequence
  GPC3A-057 VL
EIVLTQSPSVSVAPGKTARITCGGNNIGSKSVHWYQQKPGQAPVLVIYYDSDRPSGIPERFSGSNSGNTATLTISRVEAGDEADYYCQVWDSSSDHVVFGGGTKVEIKR

SEQ ID NO: 381 - protein, 108 aa, Artificial Sequence
  GPC3A-058 VL
QSVLTQPPSVSVAPGKTARITCGGNNIGSKSVHWYQQKPGQAPVLVVYDDSDRPSGIPERFSGSNSGNTATLTISRVEAGDEADYYCQVWDSSSDHVFGTGTKVTVLG

SEQ ID NO: 382 - protein, 108 aa, Artificial Sequence
  GPC3A-059 VL
SYVLTQPPSVSVAPGKTARITCGGNNIGSKSVYWYQQKPGQAPVLVIYYDSDRPSGIPERFSGSNSGNTATLTISRVEAGDEADYYCQVWDSSSDHVFGTGTKVTVLG

SEQ ID NO: 383 - protein, 107 aa, Artificial Sequence
  GPC3A-060 VL
SYVLTQPPSVSVAPGKTARLTCGGNNIGSESVHWYQQKPGQAPLLVVYDDDDRPSGIPERFSGSNSEDTATLTISGTQALDEAEYYCQTWDSSTAIFGTGTKLTVLG

SEQ ID NO: 384 - protein, 109 aa, Artificial Sequence; identical to SEQ ID NO: 378
  GPC3A-061 VL

SEQ ID NO: 385 - protein, 113 aa, Artificial Sequence
  GPC3A-062 VL
QSVLTQPPSVSGAPGQRVTISCTGSSSNIGAGYDVHWYQQLPGTAPKLLIYGNSNWPSGVPDRFSGSKSGTSASLAITGLRAEDEADYYCQSYDSSLSGSYVFGTGTKVTVLG

SEQ ID NO: 386 - protein, 111 aa, Artificial Sequence
  GPC3A-063 VL
QTVVTQPPSASGTPGQRVTISCSGSWSNIGSYTVNWYQHLPGTAPKLLISGNNQRPSGVPGRFSGSKSGTSASLAISGLQSEDEADYHCAAWDDNLNGVVFGGGTKLTVLG

SEQ ID NO: 387 - protein, 109 aa, Artificial Sequence
  GPC3A-064 VL
LPVLTQPPSLSVAPGKTARLTCGGNNIGSKSVHWYHQKPGQAPVLVVYDDTDRPSGIPERFSGSNSGNTAALTISRVEVGDEADYYCQVWDRSSAHWVFGGGTKLTVLG

SEQ ID NO: 388 - protein, 109 aa, Artificial Sequence; identical to SEQ ID NO: 361
  GPC3A-067 VL

SEQ ID NO: 389 - protein, 111 aa, Artificial Sequence
  GPC3B-54 VL
QSVLTQPPSASGTPGQRVTISCSGSNSNIGSDTVNWYQQLPGTAPKLLIYRDNQRPSGVPDRFSGSKSGTSASLAISGLQSEDEADYYCTTWDDSLNGLVFGGGTKVTVLG

SEQ ID NO: 390 - protein, 109 aa, Artificial Sequence
  GPC3B-60 VL
SYVLTQPPSVSVSPGQTATIACSGDNLENKFVYWYHQKPGQSPVLVMYEDNKRPSGIPERFSGSNSGNTAALTISGAQPMDEADYYCQTWDSPTGLFVFGTGTKVTVLG

SEQ ID NO: 391 - protein, 113 aa, Artificial Sequence
  GPC3B-63 VL
EIVLTQSPLSLPVTPGEPASISCRSSQSLLHSNGYNYLDWYLQKPGQSPQLLIYLGSNRASGVPDRFSGSGSGTDFTLKISRVEAEDVGVYYCMQALQTPPTFGQGTKVEIKR

SEQ ID NO: 392 - protein, 110 aa, Artificial Sequence
  GPC3B-66 VL
QAVLTQPPSVSVAPGKTASITCGGNNIGSKSVHWYQQKPGQAPVLVIYYDSDRPSGIPERFSGSNSGNTATLTISRVEAGDEADYYCQVWDSSSDHLYVFGTGTKVTVLG

SEQ ID NO: 393 - protein, 111 aa, Artificial Sequence
  GPC3B-68 VL
QSVLTQPPSVSAAPGQKVTISCSGSSSNIGNNYVSWYQQLPGTAPKLLIYDNIKRPSGIPDRFSGSKSGTSATLGITGLQTGDEADYYCGTWDSSLSAGVFGGGTKLTVLG

SEQ ID NO: 394 - protein, 109 aa, Artificial Sequence
  GPC3B-71 VL
SYVLTQPPSVSVAPGKTARVTCGGNNIGSKSVHWYQQKPGQAPVLVMYYDSDRPSGIPERFSGSNSGNTATLTISSVEAGDEADYYCQVWDSSSDHYVFGTGTKVTVLG

SEQ ID NO: 395 - protein, 111 aa, Artificial Sequence
  GPC3B-76 VL
QSVVTQPPSVSAAPGQKVTISCSGSSSNIGNNYVSWYQQLPGTAPKLLIYDNNKRPSGIPDRFSGSKSGTSATLGITGLQTGDEAAYYCGTWDSSLSAGVFGTGTKVTVLG

SEQ ID NO: 396 - protein, 107 aa, Artificial Sequence
  GPC3B-78 VL
LPVLTQPPSVSVSPGQTASITCSGDKLGDKYAYWYQQKPGQSPVLVIYQDNKRPSGIPERFSGSNSGNTATLTISGTQAMDAADYYCQTWDRSTYVFGTGTKVTVLG

SEQ ID NO: 397 - protein, 112 aa, Artificial Sequence
  GPC3B-80 VL
QAVLTQPPSASGTPGQRVTISCSGSSSNIGSNTVNWYQQLPGTAPKLLIYSNNQRPSGVPDRFSGSKSGTSAYLAISGLQSEDEADYYCAAWDDSLNGWGVFGGGTKLTVLG

SEQ ID NO: 398 - protein, 110 aa, Artificial Sequence
  GPC3B-81 VL
SYELTQPPSVSVAPGKTARITCGGNNIGSKSVHWYQQKPGQAPVLVIYYDSDRPSGIPERFSGSNSGNTATLTISRVEAGDEADYYCQVWDSSSDLLYVFGTGTKVTVLG

SEQ ID NO: 399 - protein, 112 aa, Artificial Sequence
  GPC3B-82 VL
QSVLTQPPSVSGAPGQRVTISCTGSSSNIGAGFDVHWYQQLPGTAPKLLIYDNNNRPSGVPDRFSGSKSDTSASLAITGLQAEDEADYYCQSFDSSLSGWVFGGGTKLTVLG

SEQ ID NO: 400 - protein, 111 aa, Artificial Sequence
  GPC3B-85 VL
QAVLTQPPSASGTPGQRVTISCSGSSSNIGSNTVNWYQQLPGTAPKLLIYSNNQRPSGVPDRFSGSKSGTSASLAISGLQSEDEADYYCAAWDDSLNGYVFGTGTKVTVLG

SEQ ID NO: 401 - protein, 113 aa, Artificial Sequence
  GPC3B-87 VL
DVVMTQSPLSLPVTPGEPASVSCRSSQSLLHSNGYNYLDWYLQKPGQSPQLLIYLGSNRASGVPDRFSGSGSGTDFTLKISRVEAEDVGVYYCMQALQTPWTFGQGTKVEIKR

SEQ ID NO: 402 - protein, 108 aa, Artificial Sequence
  GPC3B-92 VL
QSVLTQPPSVSVSPGQTARITCSGETLAKRYAHWYQQKPGQAPVLLIYRDTERPSGIPERFSGSSSGTTITLTITGVQAEDEADYYCQSADNSRTFVFGPGTKVTVLG

SEQ ID NO: 403 - protein, 111 aa, Artificial Sequence
  GPC3B-93 VL
NFMLTQPHSVSESPGKTVTISCTGSSGSIASNYVQWYQQRPGSAPTTVIYEDNQRPSGVPDRFSGSIDSSSNSASLTISGLKTEDEADYYCQSYDSSNWVFGGGTKLTVLG

SEQ ID NO: 404 - protein, 111 aa, Artificial Sequence
  GPC3B-110 VL
QSVLTQPPSASGTPGQRVTVSCSGSSSNIGSNTVNWYQQLPGTAPKLLLYSSNQRPSGVPDRFSGSRSGTSASLAISGLQSEDEADYYCAAWDDSLNGPVFGGGTKLTVLG

SEQ ID NO: 405 - protein, 111 aa, Artificial Sequence
  GPC3B-113 VL
SYELTQPPSASGTPGQRVTISCSGSSSNIGSNSVSWYQHLPGVAPKLLIYSNNQRPSGVPDRFSGSKTGTSASLAISGLQSEDEGDYYCAAWDDSLNGVLFGGGTKLTVLG

SEQ ID NO: 406 - protein, 110 aa, Artificial Sequence
  GPC3B-115 VL
SYELTQPPSVSVAPGKTARITCGGNNIGSKSVHWYQQKPGQAPVLVVYDDSDRPSGIPERFSGSNSGNTATLTISRVEAGDEADYYCQVWDSSSDPLYVFGTGTKVTVLG

SEQ ID NO: 407 - protein, 111 aa, Artificial Sequence
  GPC3B-119 VL
QSVVTQPPSVSAAPGQKVTISCSGSSSNIGNNYVSWYQQIPGTAPKLLIYDNNKRPSGIPDRFSGSRSGTSATLGITGLQTGDEAHYYCATWDNSLSALIFGGGTKVTVLG

SEQ ID NO: 408 - protein, 111 aa, Artificial Sequence
  GPC3B-125 VL
QSALTQPASVSGSPGQSITISCTGTSSDVGGYNYVSWFQQHPGKAPKLIIYEVSNRPSGVSDRFSGSKSGSTASLTISGLQAEDEANYYCSSYTSSTTVIFGGGTKLTVLG

SEQ ID NO: 409 - protein, 248 aa, Artificial Sequence
  GPC3A-034 scFv
QPVLTQPPSASGTPGQRVTISCSGSSSNIGSNNVIWYQQLPGAAPKLLIYSNHRRPSGVPDRFSGSRSGTSASLAISGLQSEDEADYYCAAWDDSLDGYLFGTGTKVTVLGSRGGGGSGGGGSGGGGSLEMAQVQLQQWGAGLLKPSETLSLTCAVYGGSFSGYYWSWIRQPPGKGLEWIGEINHSGSTNYNPSLKSRVTISVDTSKNQFSLELSSVTAADTAVYYCARGYGGRFDYWGQGTLVTVSS

SEQ ID NO: 410 - protein, 249 aa, Artificial Sequence
  GPC3A-035 scFv
QAVLTQPPSASQTPGQMVTISCSGTSSNIGSNYVFWYQQLPGTAPKLLIYKNFQRPSGVPGRFSGSKSGTAASLAISGLRSEDEADYFCAAWDDALSGYVFGAGTKVTVLGSRGGGGSGGGGSGGGGSLEMAQVQLVQSGAEVKKPGASVKVSCKASGYTFTGYYMHWVRQAPGQGLEWMGWINPNSGGTNYAQKFQGRVTMTRDTSISTAYMELSRLRSDDTAVYYCARSWTSGFDYWGQGTLVTVSS

SEQ ID NO: 411 - protein, 250 aa, Artificial Sequence
  GPC3A-037 scFv
QSVLTQPPSVSAAPGQRVTISCSGTRSNIGSDYVSWYQHLPGTAPKLLVYGDNLRPSGIPDRFSASKSGTSATLGITGLQTGDEADYYCGTWDYTLNGVVFGGGTKLTVLGSRGGGGSGGGGSGGGGSLEMAQVQLVESGGGLVQPGGSLRLSCAASGFTFSSYAMSWVRQAPGKGLEWVSVIYSGGSSTYYADSVKGRFTISRDNSKNTLYLQMNSLRAEDTAVYYCARTSYLNHGDYWGQGTLVTVSS

SEQ ID NO: 412 - protein, 246 aa, Artificial Sequence
  GPC3A-038 scFv
QSVLTQPPSVSVAPGKTARITCGGNNIGSKSVHWYQQKPGQAPVLVIYYDSDRPSGIPERFSGSNSGNTATLTISRVEAGDEADYYCQVWDSSSDHVVFGGGTKLTVLGSRGGGGSGGGGSGGGGSLEMAQVQLVQSGAEVKKPGASVKVSCKASGYTFTSYYMHWVRQAPGQGLEWMGIINPSGGSTSYAQKFQGRVTMTRDTSTSTVYMELSSLRSEDTAVYYCARKVTGYDSWGQGTLVTVSS

SEQ ID NO: 413 - protein, 246 aa, Artificial Sequence
  GPC3A-039 scFv
SYVLTQPPSVSVAPGKTARITCGGNNIGSKSVHWYQQKPGQAPVLVIYYDSDRPSGIPERFSGSNSGNTATLTISRVEAGDEADYYCQVWDSSSDHWVFGGGTKLTVLGSRGGGGSGGGGSGGGGSLEMAQVQLVQSGGGLVHPGGSLRLSCAGSGFTFSSYAMHWVRQAPGKGLEWVSAIGTGGGTYYADSVKGRFTISRDNAKNSLYLQMNSLRAEDTAVYYCARYGRKSIDAWGQGTLVTVSS

SEQ ID NO: 414 - protein, 249 aa, Artificial Sequence
  GPC3A-040 scFv
LPVLTQPPSASGTPGQRVTISCSGSSSNIGSNYVYWYQQLPGTAPKLLIYSNNQRPSGVPDRFSGSKSGTSASLAISGLRSEDEADYYCAAWDDSLSGYVFGTGTKVTVLGSRGGGGSGGGGSGGGGSLEMAQVQLVQSGAEVKKPGASVTVSCKASGYTFTGYYMHWVRQAPGQGLEWMGWINPNSGGTNYAQKFQGRVTMTRDTSISTAYMELSRLRSDDTAVYYCARRGYYGYDSWGQGTLVTVSS

SEQ ID NO: 415 - protein, 249 aa, Artificial Sequence
  GPC3A-041 scFv
QAVLTQPPSASQTPGQMVTISCSGTSSNIGSNYVFWYQQLPGTAPKLLIYKNFQRPSGVPGRFSGSKSGTAASLAISGLRSEDEADYFCAAWDDALSGYVFGAGTKVTVLGSRGGGGSGGGGSGGGGSLEMAEVQLVQSGAEVKKPGASVKVSCKASGYTFTGYYMHWVRQAPGQGLEWMGWINPNSGGTNYAQKFQGRVTMTRDTSISTAYMELSRLRSDDTAMYYCARSGKYYGDKWGQGTLVTVSS

SEQ ID NO: 416 - protein, 249 aa, Artificial Sequence
  GPC3A-042 scFv
SYVLTQPPSASGTPGQRVTISCFGSSSDIGSNSVFWYQQLPGAAPKLLIYSTQYRPSGVPDRFSGSKSGTSASLAISGLQSEDEAEYHCATWDDSLNGYVFGSGTKVTVLGSRGGGGSGGGGSGGGGSLEMAQVQLQQSGAEVKKPGASVKVSCKASGYSFTGYYVYWMRQAPGKGLEWMGWMNPRSGGTNYAQKFQGRVTMTRDTSISTAYMELSRLTSDDTAVYYCARSSYYWADSWGQGTLVTVSS

SEQ ID NO: 417 - protein, 256 aa, Artificial Sequence
  GPC3A-043 scFv
QSVLTQPPSASGTPGQRVTISCSGSSSNIGTNYVYWYQQLPGTAPKLIIYRNNQRPSGVPDRFSGSESGTSASLAISGLRSEDEADYYCAVWDDSLSGVVFGGGTKLTVLGSRGGGGSGGGGSGGGGSLEMAEVQLVQSGAEVKKPGATVKVSCKVSGYTFTDYYMHWVQQAPGKGLEWMGLVDPEDGETIYAEKFQGRVTITADTSTDTAYMELSSLRSEDTAVYYCARELRDVAYYPWGVEDFWGQGTLVTVSS

SEQ ID NO: 418 - protein, 246 aa, Artificial Sequence
  GPC3A-044 scFv
SYVLTQPPSVSVAPGKTARITCGGDNIGYKGVHWYQQKPGQAPVLVVYDDSDRPSGIPERFSGSNSGNTATLTISRVEAGDEADYYCQVWDSSSDHVVFGGGTKLTVLGSRGGGGSGGGGSGGGGSLEMAQVQLQQWGAGLLKPSETLSLTCAVYGGSFSGYYWSWIRQPPGKGLEWIGEINHSGSTNYNPSLKSRVTISVDTSKNQFSLKLSSVTAADTAVYYCARYYVPYLSDWGQGTLVTVSS

SEQ ID NO: 419 - protein, 248 aa, Artificial Sequence
  GPC3A-045 scFv
QSVLTQPPSVSGTPGQRVIISCPGSTSNIGTNTVNWYQQFPGTAPKLLIYSNNQRPSGVPDRFSGSKSGTSASLAISGLQSEDEADYYCAAWDDSLNGVVFGGGTKLTVLGSRGGGGSGGGGSGGGGSLEMAQMQLVQSGGGLVKPGGSLRLSCAASGFTFSDYYMSWIRQAPGKGLEWVSYISSSGSTIYYADSVKGRFTISRDNAKNSLYLQMNSLRAEDTAVYYCARASDLYGDWGQGTLVTVSS

SEQ ID NO: 420 - protein, 253 aa, Artificial Sequence
  GPC3A-046 scFv
QAVLTQPPSVSGTPGQRVTISCSGSSSNFGSNTVHWYQQVPGTAPKLLIFSNTQRPSEIPDRFSGSKSGTSASLAISGLQSEDEADYYCAAWDDSLTGVVFGGGTKLTVLGSRGGGGSGGGGSGGGGSLEMAQVQLVQSGAEVKKPGASVTVSCKASGYRFSNYGVSWVRQAPGQGLEWMGWISGSNGNTNYAQKFLGRVTMTTDTSTTTAYMELSSLRSDDTAVYYCARGNRRYYSPIIDPWGQGTLVTVSS

SEQ ID NO: 421 - protein, 250 aa, Artificial Sequence
  GPC3A-047 scFv
LPVLTQPPSASGTPGQRVTISCSGSRSNIASNDVYWYQQLPGTAPKRLIYKKNQRPSGVPDRFSASKSGTSASLAISGLRSEDEADYYCAAWDDNLSGYVFGTGTKVTVLGSRGGGGSGGGGSGGGGSLEMAQVQLVQSGAEVKKPGASVKVSCKAPGYTFTGYYMHWVRQAPGQGLEWMGWINPNSGGTNYAQKFQGRVTMTRDTSISTAYMELSRLRSDDTAVYYCARSDYGSLYDKWGQGTLVTVSS

SEQ ID NO: 422 - protein, 247 aa, Artificial Sequence
  GPC3A-048 scFv
QPVLTQPPSVSVAPGKTARITCGGNNIGSKSVHWYQQKPGQAPVLVIYYDSDRPSGIPERFSGSNSGNTATLTISRVEAGDEADFYCQVWDSSSDRGVFGGGTKLTVLGSRGGGGSGGGGSGGGGSLEMAEVQLVESGGGEVQPGRSLRLSCAASGFTFSSYAMHWVRQAPGKGLEWVAVISYDGSNKYYADSVKGRFTISRDNSKNTLYLQMNSLRAEDTAVYYCARSSFVATDYWGQGTLVTVSS

SEQ ID NO: 423 - protein, 253 aa, Artificial Sequence
  GPC3A-049 scFv
QAVLTQPSSASGTPGQRVTISCSGGSSNIGSNYVYWYQQLPGTAPKLLIYRNNQRPSGVPDRFSGSKSGTSASLAISGLRSEDEADYYCAAWDDSLSGWVFGGRTKLTVLGSRGGGGSGGGGSGGGGSLEMAQVQLVQSGAEVKEPGASVKVSCKASGYTFTGYYMHWVRQAPGQGLEWMGWINPNSGGTNYAQKFQGRVTMTRDTSISTAYMELSRLRSDDTAVYYCARHGGIGSMRSFDQWGQGTLVTVSS

SEQ ID NO: 424 - protein, 249 aa, Artificial Sequence
  GPC3A-050 scFv
QAVLTQPSSASGTPGQRVTISCSGSSSNIGSNTVNWYQQLPGTAPKLLIYSNNQRPSGVPDRFSGSKSGTSASLAISGLQSEDEADYYCAAWDDSLNGPVFGTGTKVTVLGSRGGGGSGGGGSGGGGSLEMAQITLKESGAEVKKPGASVKVSCKASGYSFTGYYVYWMRQAPGKGLEWMGWMNPRSGGTNYAQKFQGRVTMTRDTSISTAYMELSRLTSDDTATYYCARSGYRWLDVWGQGTLVTVSS

SEQ ID NO: 425 - protein, 254 aa, Artificial Sequence
  GPC3A-051 scFv
QAVLTQPSSASGAPGQRVTISCTGGSSNIGAGYDVHWYQQLPGTAPKLLIYGNSNRPSGVPDRFSGSKSGTSASLAITGLQAEDEADYYCQSYDSSLSGYVFGTGTKVTVLGSRGGGGSGGGGSGGGGSLEMAQVQLVQSGAEVKKPGSSVKVSCKASGGAFSSYAISWVRQAPGQGLEWMGGIIPIFGTANYAQKFQGRVTITADESTSTAYMELSSLRSEDTAVYYCARMLYLSGRYYWDSWGQGTLVTVSS

SEQ ID NO: 426 - protein, 249 aa, Artificial Sequence
  GPC3A-052 scFv
QAVLTQPSSASGTPGQRVTISCSGSSSNIGSNYVYWYQQLSGTAPKLLIYRNNQRPSGVPDRFSGSKSGTSASLAISGLRSEDEADYYCAAWDDSLSGYVFGTGTKVTVLGSRGGGGSGGGGSGGGGSLEMAEVQLVESGAEVKKPGASVKVSCKASGYTFTGYYMHWVRQAPGQGLEWMGWINPNSGGTNYAQKFQGRVTMTRDTSISTAYMELSRLRSDDTAVYYCARSHSSGYDKWGQGTLVTVSS

SEQ ID NO: 427 - protein, 251 aa, Artificial Sequence
  GPC3A-053 scFv
QSVLTQPPSASAAPGQRVTISCSGTSSNIGSNYVWWYQQLPGAAPRLLIYGNSNRPSGVPDRFSGSKSGTSASLAITGLQAEDEADYYCQSYDSSLSGSNVFGTGTKVTVLGSRGGGGSGGGGSGGGGSLEMAQLQLQESGPGLVKPSETLSLTCTVSGGSISSSSYYWGWIRQPPGKGLEWIGSIYYSGSTYYNPSLKSRVTISVDTSKNQFSLKLSSVTAADTAVYYCARWWSGSYDTWGQGTLVTVSS

SEQ ID NO: 428 - protein, 251 aa, Artificial Sequence
  GPC3A-054 scFv
SYELTQPPSASGTPGQRVTISCSGSSSNIGSNYVYWYQQLPGTAPKLLIYRNNQRPSGVPDRFSGSKSGTSASLAISGLRSEDEADYYCAAWDDSLSGYVFGTGTKVTVLGSRGGGGSGGGGSGGGGSLEMAQMQLVQSGAEVKKPGASVKVSCKASGYTFTSYGISWVRQAPGQGLEWMGWISAYNGNTNYAQKLQGRVTMTTDTSTSTAYMELRSLRSDDTAVYYCARIPMYSGSSDYWGQGTLVTVSS

SEQ ID NO: 429 - protein, 247 aa, Artificial Sequence
  GPC3A-055 scFv
QPVLTQPPSVSVAPGKTARITCGGNNIGSKSVHWYQQKPGQAPVLVIYYDSDRPSGIPERFSGSNSGNTATLTISRVEAGDEADYYCQVWDSSSDHYVFGTGTKVTVLGSRGGGGSGGGGSGGGGSLEMAQVQLVQSGAEVKKPGASVKVSCKASGYTFTSYYMHWVRQAPGQGLEWMGIINPSGGSTSYAQKFQGRVTMTRDTSTSTVYMELSSLRSEDTAVYYCARWHGGPYDYWGQGTLVTVSS

SEQ ID NO: 430 - protein, 251 aa, Artificial Sequence
  GPC3A-056 scFv
DIQLTQSPSSLSASVGDRVTITCRASQSISSYLNWYQQKPGKAPKLLIYAASSLQSGVPSRFSGSGSGTDFTLTISSLQPEDFATYYCQQSYSTPITFGQGTRLEIKRSRGGGGSGGGGSGGGGSLEMAQVQLQQSGAEVKKFGASVKVSCKASGYSFNDYYIHWVRQAPGQGLEWMGWINPNNGDTKYEKKWQGRVTMTRDTSITTAYMELSSLRSDDTAVYYCARFSTHNWWWPTYDYWGQGTLVTVSS

SEQ ID NO: 431 - protein, 250 aa, Artificial Sequence
  GPC3A-057 scFv
EIVLTQSPSVSVAPGKTARITCGGNNIGSKSVHWYQQKPGQAPVLVIYYDSDRPSGIPERFSGSNSGNTATLTISRVEAGDEADYYCQVWDSSSDHVVFGGGTKVEIKRSRGGGGSGGGGSGGGGSLEMAEVQLVESGGGLIQPGGSLRLSCAASGFTFSSYAMSWVRQAPGKGLEWVSAISGSGGSTYYADSVKGRFTISRDNSKNTLYLQMNSLRAEDTAVYYCARYNYMSSGFYDRWGQGTLVTVSS

SEQ ID NO: 432 - protein, 249 aa, Artificial Sequence
  GPC3A-058 scFv
QSVLTQPPSVSVAPGKTARITCGGNNIGSKSVHWYQQKPGQAPVLVVYDDSDRPSGIPERFSGSNSGNTATLTISRVEAGDEADYYCQVWDSSSDHVFGTGTKVTVLGSRGGGGSGGGGSGGGGSLEMAQVQLVQSGADVRKPGASVKVSCKASGYTFASHGISWVRQAPGQGLEWLGWISPYTGNTNYAQKFQGRVTMATDTSTSTAYMELRSLRSDDTAIYYCARGKRTLASCFDYWGQGTLVTVSS

SEQ ID NO: 433 - protein, 246 aa, Artificial Sequence
  GPC3A-059 scFv
SYVLTQPPSVSVAPGKTARITCGGNNIGSKSVYWYQQKPGQAPVLVIYYDSDRPSGIPERFSGSNSGNTATLTISRVEAGDEADYYCQVWDSSSDHVFGTGTKVTVLGSRGGGGSGGGGSGGGGSLEMAQVQLVQSGAEVKKPGASVTVSCKASGYTFTRYGITWVRQAPGQGLEWMGWISAYSDKTNYAQKLQGRVTMTTDISTNTAYMELSSLRSEDTAVYYCARSRWSYMDVWGQGTLVTVSS

SEQ ID NO: 434 - protein, 247 aa, Artificial Sequence
  GPC3A-060 scFv
SYVLTQPPSVSVAPGKTARLTCGGNNIGSESVHWYQQKPGQAPLLVVYDDDDRPSGIPERFSGSNSEDTATLTISGTQALDEAEYYCQTWDSSTAIFGTGTKLTVLGSRGGGGSGGGGSGGGGSLEMAQVQLVQSGGEVKKPGASVKVSCKASGYTFNSYAISWVRQAPGQGLEWMGWISAYNGNTNYAQKLQGRVTMTTDTSTNTAFMELRSLRSDDTAVYYCAREGYGSWAMDQWGQGTLVTVSS

SEQ ID NO: 435 - protein, 247 aa, Artificial Sequence
  GPC3A-061 scFv
QPVLTQPPSVSVAPGKTARITCGGNNIGSKSVHWYQQKPGQAPVLVIYYDSDRPSGIPERFSGSNSGNTATLTISRVEAGDEADYYCQVWDSSSDHYVFGTGTKVTVLGSRGGGGSGGGGSGGGGSLEMAQVQLVQSGAEVKKPGASVKVSCKASGYTFTSYGISWVRQTPGQGLEWMGWISAYNGNTNYAQKLQGRVTMTTDTSTSTAYMELSSLRSEDTAVYYCARKGSSQFDQWGQGTLVTVSS

SEQ ID NO: 436 - protein, 257 aa, Artificial Sequence
  GPC3A-062 scFv
QSVLTQPPSVSGAPGQRVTISCTGSSSNIGAGYDVHWYQQLPGTAPKLLIYGNSNWPSGVPDRFSGSKSGTSASLAITGLRAEDEADYYCQSYDSSLSGSYVFGTGTKVTVLGSRGGGGSGGGGSGGGGSLEMAQMQLVQSGSELKKPGASVKVSCKASGGTFSSYAISWVRQAPGQGLEWMGGIIPKIGTANYAQKFQGRVTITADESTSTAYMELSSLRSEDTAMYYCARMYMDMGWGWGYWDWWGQGTLVTVSS

SEQ ID NO: 437 - protein, 251 aa, Artificial Sequence
  GPC3A-063 scFv
QTVVTQPPSASGTPGQRVTISCSGSWSNIGSYTVNWYQHLPGTAPKLLISGNNQRPSGVPGRFSGSKSGTSASLAISGLQSEDEADYHCAAWDDNLNGVVFGGGTKLTVLGSRGGGGSGGGGSGGGGSLEMAQVQLVQSGAEVKKPGASVKVSCKASGYTFTSYYMHWVRQAPGQGLEWMGIINPSGGSASYAQKFQGRVTMTRDTSTSTVYMELSSLRSEDTAVYYCARDRLASDAFDIWGQGTMVTVSS

SEQ ID NO: 438 - protein, 250 aa, Artificial Sequence
  GPC3A-064 scFv
LPVLTQPPSLSVAPGKTARLTCGGNNIGSKSVHWYHQKPGQAPVLVVYDDTDRPSGIPERFSGSNSGNTAALTISRVEVGDEADYYCQVWDRSSAHWVFGGGTKLTVLGSRGGGGSGGGGSGGGGSLEMAQMQLVQSGAEVKKPGASVKVSCKASGYTFTIYGISWVRQAPGQGLEWMGWISPYNDNTIYAQKVQGRVTMTTDTSTSTAYMELRSLRSDDTAVYYCARMGVGWGYAQDSWGQGTLVTVSS

SEQ ID NO: 439 - protein, 246 aa, Artificial Sequence
  GPC3A-067 scFv
QSVLTQPPSVSVAPGKTARITCGGNNIGSKSVHWYQQKPGQAPVLVIYYDSDRPSGIPERFSGSNSGNTATLTISRVEAGDEADYYCQVWDSSSDHVVFGGGTKLTVLGSRGGGGSGGGGSGGGGSLEMAEVQLVQSGAEVKKPGSSVKVSCKASGGTFSSYAISWVRQAPGQGLEWMGRIIPIFGITNYAQKFQGRVTITADKSTSTAYMELSSLRSEDTAVYYCARGAEMSDYWGQGTLVTVSS

SEQ ID NO: 440 - protein, 252 aa, Artificial Sequence
  GPC3B-54 scFv
QSVLTQPPSASGTPGQRVTISCSGSNSNIGSDTVNWYQQLPGTAPKLLIYRDNQRPSGVPDRFSGSKSGTSASLAISGLQSEDEADYYCTTWDDSLNGLVFGGGTKVTVLGSRGGGGSGGGGSGGGGSLEMAEVQLVQSGAEVKKPGASVKLSCKTSGYTFIDYYVYWVRQAPGQGLEWMGGIIPIFGTANYAQKFQGRVTITADKSTSTAYMELSSLGSEDTAVYYCARERRYSSSPSDHWGQGTLVTVSS

SEQ ID NO: 441 - protein, 249 aa, Artificial Sequence
  GPC3B-60 scFv
SYVLTQPPSVSVSPGQTATIACSGDNLENKFVYWYHQKPGQSPVLVMYEDNKRPSGIPERFSGSNSGNTAALTISGAQPMDEADYYCQTWDSPTGLFVFGTGTKVTVLGSRGGGGSGGGGSGGGGSLEMAEVQLVESGAEVKKPGASVKVSCKASGYTFTSYYMHWVRQAPGQGLEWMGIINPSGGSTSYAQKFQGRVTMTRDTSTSTVYMELSSLRSEDTAVYYCARSLYSQPYIDGWSQGTLVTVSS

SEQ ID NO: 442 - protein, 256 aa, Artificial Sequence
  GPC3B-63 scFv
EIVLTQSPLSLPVTPGEPASISCRSSQSLLHSNGYNYLDWYLQKPGQSPQLLIYLGSNRASGVPDRFSGSGSGTDFTLKISRVEAEDVGVYYCMQALQTPPTFGQGTKVEIKRSRGGGGSGGGGSGGGGSLEMAQVQLVQSGAEVKKPGASVKVSCKASGYTFTSYYMHWVRQAPGQGLEWMGIINPSGGSTSYAQKFQGRVTMTRDTSTSTVYMELSSLRSEDTAVYYCARSLHAMRWSQTMDSWGQGTLVTVSS

SEQ ID NO: 443 - protein, 249 aa, Artificial Sequence
  GPC3B-66 scFv
QAVLTQPPSVSVAPGKTASITCGGNNIGSKSVHWYQQKPGQAPVLVIYYDSDRPSGIPERFSGSNSGNTATLTISRVEAGDEADYYCQVWDSSSDHLYVFGTGTKVTVLGSRGGGGSGGGGSGGGGSLEMAQVQLVQSGAEVKRPGASVKVSCKASGYTFIGQYLHWVRQAPGQGLEWMGRINPMTGVTNYAPKFQGRVTMTRDTSISTGYMEISRLRSDDTAVYYCARFSSGYSRDTWGQGTLVTVSS

SEQ ID NO: 444 - protein, 249 aa, Artificial Sequence
  GPC3B-68 scFv
QSVLTQPPSVSAAPGQKVTISCSGSSSNIGNNYVSWYQQLPGTAPKLLIYDNIKRPSGIPDRFSGSKSGTSATLGITGLQTGDEADYYCGTWDSSLSAGVFGGGTKLTVLGSRGGGGSGGGGSGGGGSLEMAQVQLVQSGAEVKKPGSSVKVSCKASGGTFSSYAISWVRQAPGQGLEWMGRIIPILGIANYAQKFQGRVTITADKSTSTAYMELSSLRSEDTAVYYCARYGYEGHDTWGQGTLVTVSS

SEQ ID NO: 445 - protein, 250 aa, Artificial Sequence
  GPC3B-71 scFv
SYVLTQPPSVSVAPGKTARVTCGGNNIGSKSVHWYQQKPGQAPVLVMYYDSDRPSGIPERFSGSNSGNTATLTISSVEAGDEADYYCQVWDSSSDHYVFGTGTKVTVLGSRGGGGSGGGGSGGGGSLEMAEVQLVESGGGLVKPGGSLRLSCAASGFTFSRYTMNWVRQAPGKGLEWVSSISSSGSYIYYADSVKGRFTISRDNAKNSLFLQMDSLRAEDTAVYYCARQGHMWYVPVDAWGQGTLVTVSS

SEQ ID NO: 446 - protein, 244 aa, Artificial Sequence
  GPC3B-76 scFv
QSVVTQPPSVSAAPGQKVTISCSGSSSNIGNNYVSWYQQLPGTAPKLLIYDNNKRPSGIPDRFSGSKSGTSATLGITGLQTGDEAAYYCGTWDSSLSAGVFGTGTKVTVLGSRGGGGSGGGGSGGGGSLEMAQMQLVQSGAEVKEPGASVKVSCKASGYTFTDYYIHWVRQAPGQGLEWMGWINPNSGGTNYAQKFQGRVTMTRDTSISTAYMELSRLRSDDTAVYYCARNYDWGQGTLVTVSS

SEQ ID NO: 447 - protein, 245 aa, Artificial Sequence
  GPC3B-78 scFv
LPVLTQPPSVSVSPGQTASITCSGDKLGDKYAYWYQQKPGQSPVLVIYQDNKRPSGIPERFSGSNSGNTATLTISGTQAMDAADYYCQTWDRSTYVFGTGTKVTVLGSRGGGGSGGGGSGGGGSLEMAQMQLVQSGAEVKKPGASVKVSCKASGYTFTSYYMHWVRQAPGQGLEWMGIINPSGGSTSYAQKFQGRVTMTRDTSTSTVYMELSSLRSEDTAVYYCARGYSSFFDSWGQGTLVTVSS

SEQ ID NO: 448 - protein, 255 aa, Artificial Sequence
  GPC3B-80 scFv
QAVLTQPPSASGTPGQRVTISCSGSSSNIGSNTVNWYQQLPGTAPKLLIYSNNQRPSGVPDRFSGSKSGTSAYLAISGLQSEDEADYYCAAWDDSLNGWGVFGGGTKLTVLGSRGGGGSGGGGSGGGGSLEMAQVQLVQSGAEVKKPGSSVKVSCKASGGTLSRFAISWVRQAPGQGLEWMGGIIPIFRTANYAQKFQGRVTITADESTSTAYMELSSLRSEDTAVYYCARMSKYYGSYSSYDEWGQGTLVTVSS

SEQ ID NO: 449 - protein, 245 aa, Artificial Sequence
  GPC3B-81 scFv
SYELTQPPSVSVAPGKTARITCGGNNIGSKSVHWYQQKPGQAPVLVIYYDSDRPSGIPERFSGSNSGNTATLTISRVEAGDEADYYCQVWDSSSDLLYVFGTGTKVTVLGSRGGGGSGGGGSGGGGSLEMAEVQLVQSGAEVKKPGASVKVSCKASGYTFTGYYMHWVRQAPGQGLEWMGRINPNSGGTNYAQKFQGRVTMTRDTSISTAYMELSRLRSDDTAVYYCARGLWDSWGQGTLVTVSS

SEQ ID NO: 450 - protein, 254 aa, Artificial Sequence
  GPC3B-82 scFv
QSVLTQPPSVSGAPGQRVTISCTGSSSNIGAGFDVHWYQQLPGTAPKLLIYDNNNRPSGVPDRFSGSKSDTSASLAITGLQAEDEADYYCQSFDSSLSGWVFGGGTKLTVLGSRGGGGSGGGGSGGGGSLEMAEVQLVQSGAEVKKPGESLKISCKGSGYSFTSYYMHWVRQAPGQGLEWMGIINPSGGSTSYAQKFQGRVTMTRDTSTSTVYMEMSSLRSEDTAVYYCARYPVYMETSDFDSWGSRYSGDRLL

SEQ ID NO: 451 - protein, 257 aa, Artificial Sequence
  GPC3B-85 scFv
QAVLTQPPSASGTPGQRVTISCSGSSSNIGSNTVNWYQQLPGTAPKLLIYSNNQRPSGVPDRFSGSKSGTSASLAISGLQSEDEADYYCAAWDDSLNGYVFGTGTKVTVLGSRGGGGSGGGGSGGGGSLEMAQVQLVQSGSELKKPGASVKVSCKASGYTFTSYAMNWVRQAPGQGLEWMGWINTNTGNPTYAQGFTGRFVFSLDTSVSTAYLQISSLKAEDTAVYYCARSSLYWMGSKWSRQTDMWGQGTLVTVSS

SEQ ID NO: 452 - protein, 247 aa, Artificial Sequence
  GPC3B-87 scFv
DVVMTQSPLSLPVTPGEPASVSCRSSQSLLHSNGYNYLDWYLQKPGQSPQLLIYLGSNRASGVPDRFSGSGSGTDFTLKISRVEAEDVGVYYCMQALQTPWTFGQGTKVEIKRSRGGGGSGGGGSGGGGSLEMAEVQLVQSGAEVRKPGSSVKVSCQASGGTFGSYAISWVRQAPGQGLEWMGRIIPVLGRTKYAQKFQGRVTVTADTSTSTVYMELTSLTSEDTAVYYCARTNDSWGQGTLVTVSS

SEQ ID NO: 453 - protein, 249 aa, Artificial Sequence
  GPC3B-92 scFv
QSVLTQPPSVSVSPGQTARITCSGETLAKRYAHWYQQKPGQAPVLLIYRDTERPSGIPERFSGSSSGTTITLTITGVQAEDEADYYCQSADNSRTFVFGPGTKVTVLGSRGGGGSGGGGSGGGGSLEMAEVQLVQSGAEVKKPGASVKVSCKASGYTFSNYYMHWVRQAPGQGLEWMGIINPSGGTTTYAQKFQGRVTMTRDTSTSTVYMELSSLRSEDTAVYYCARPSMWTSSMGDVWGQGTLVTVSS

SEQ ID NO: 454 - protein, 255 aa, Artificial Sequence
  GPC3B-93 scFv
NFMLTQPHSVSESPGKTVTISCTGSSGSIASNYVQWYQQRPGSAPTTVIYEDNQRPSGVPDRFSGSIDSSSNSASLTISGLKTEDEADYYCQSYDSSNWVFGGGTKLTVLGSRGGGGSGGGGSGGGGSLEMAEVQLVQSGAEVKKPGASVKVSCKASGYTFTSYYMHWVRQAPGQGLEWMGIINPSGGSTRYAQKFQGRVTMTRDTSTSTVYMELSSLRSEDTAVYYCARYTALKPRGIYSVDSWGQGTLVTVSS

SEQ ID NO: 455 - protein, 257 aa, Artificial Sequence
  GPC3B-110 scFv
QSVLTQPPSASGTPGQRVTVSCSGSSSNIGSNTVNWYQQLPGTAPKLLLYSSNQRPSGVPDRFSGSRSGTSASLAISGLQSEDEADYYCAAWDDSLNGPVFGGGTKLTVLGSRGGGGSGGGGSGGGGSLEMAEVQLVQSGAEVKKPGSSVKVSCQASGGTFTTYSINWVRQAPGQGLEWMGGIIPTFGTTNYAQNFQDRVTISADESTNTAYMELTSLRSEDTAVYYCARYYWRGGSGQGSVTSDYWGQGTLVTVSS

SEQ ID NO: 456 - protein, 246 aa, Artificial Sequence
  GPC3B-113 scFv
SYELTQPPSASGTPGQRVTISCSGSSSNIGSNSVSWYQHLPGVAPKLLIYSNNQRPSGVPDRFSGSKTGTSASLAISGLQSEDEGDYYCAAWDDSLNGVLFGGGTKLTVLGSRGGGGSGGGGSGGGGSLEMAQVQLVQSGAEVKKPGASVKVSCKVSGYTLTELSMHWVRQAPGKGLEWMGGFDPEDGETIYAQKFQGRVTMTEDTSTDTAYMELSSLRSEDTAVYYCARYSGDYWGQGTLVTVSS

SEQ ID NO: 457 - protein, 251 aa, Artificial Sequence
  GPC3B-115 scFv
SYELTQPPSVSVAPGKTARITCGGNNIGSKSVHWYQQKPGQAPVLVVYDDSDRPSGIPERFSGSNSGNTATLTISRVEAGDEADYYCQVWDSSSDPLYVFGTGTKVTVLGSRGGGGSGGGGSGGGGSLEMAQVQLVQSGAEVKRPGATIKVSCKTSGYTFTAYYTHWVRQAPGQGLEWVGRINANTGGTDYAPKFRDRVIMTRDTSISTAYMELGRLTSEDTAVYYCARISGYHSSGWDYWGQGTLVTVSS

SEQ ID NO: 458 - protein, 249 aa, Artificial Sequence
  GPC3B-119 scFv
QSVVTQPPSVSAAPGQKVTISCSGSSSNIGNNYVSWYQQIPGTAPKLLIYDNNKRPSGIPDRFSGSRSGTSATLGITGLQTGDEAHYYCATWDNSLSALIFGGGTKVTVLGSRGGGGSGGGGSGGGGSLEMAQVQLVQSGSELKKPGASVKVSCKASGYTFTSYAMNWVRQAPGQGLEWMGWINTNTGNPTYAQGFTGRFVFSLDTSVSTAYLQISSLKAEDTAVYYCARGYYGKYDKWGQGTLVTVSS

SEQ ID NO: 459 - protein, 246 aa, Artificial Sequence
  GPC3B-125 scFv
QSALTQPASVSGSPGQSITISCTGTSSDVGGYNYVSWFQQHPGKAPKLIIYEVSNRPSGVSDRFSGSKSGSTASLTISGLQAEDEANYYCSSYTSSTTVIFGGGTKLTVLGSRGGGGSGGGGSGGGGSLEMAQMQLVQSGSELKKPGASVKVSCKASGYTFTSYAMNWVRQAPGQGLEWMGWINTNTGNPTYAQGFTGRFVFSLDTSVSTAYLQISSLKAEDTAVYYCARQSHDEWGQGTLVTVSS

SEQ ID NO: 460 - protein, 580 aa, Artificial Sequence
  P51654 human GPC3 full-length (UNIPROT)
MAGTVRTACLVVAMLLSLDFPGQAQPPPPPPDATCHQVRSFFQRLQPGLKWVPETPVPGSDLQVCLPKGPTCCSRKMEEKYQLTARLNMEQLLQSASMELKFLIIQNAAVFQEAFEIVVRHAKNYTNAMFKNNYPSLTPQAFEFVGEFFTDVSLYILGSDINVDDMVNELFDSLFPVIYTQLMNPGLPDSALDINECLRGARRDLKVFGNFPKLIMTQVSKSLQVTRIFLQALNLGIEVINTTDHLKFSKDCGRMLTRMWYCSYCQGLMMVKPCGGYCNVVMQGCMAGVVEIDKYWREYILSLEELVNGMYRIYDMENVLLGLFSTIHDSIQYVQKNAGKLTTTIGKLCAHSQQRQYRSAYYPEDLFIDKKVLKVAHVEHEETLSSRRRELIQKLKSFISFYSALPGYICSHSPVAENDTLCWNGQELVERYSQKAARNGMKNQFNLHELKMKGPEPVVSQIIDKLKHINQLLRTMSMPKGRVLDKNLDEEGFESGDCGDDEDECIGGSGDGMIKVKNQLRFLAELAYDLDVDDAPGNSQQATPKDNEISTFHNLGNVHSPLKLLTSMAISVVCFFFLVH

SEQ ID NO: 461 - protein, 560 aa, Artificial Sequence
  Amino acids 1-560 of SEQ ID NO: 460 human GPC3 full-length (UNIPROT)
MAGTVRTACLVVAMLLSLDFPGQAQPPPPPPDATCHQVRSFFQRLQPGLKWVPETPVPGSDLQVCLPKGPTCCSRKMEEKYQLTARLNMEQLLQSASMELKFLIIQNAAVFQEAFEIVVRHAKNYTNAMFKNNYPSLTPQAFEFVGEFFTDVSLYILGSDINVDDMVNELFDSLFPVIYTQLMNPGLPDSALDINECLRGARRDLKVFGNFPKLIMTQVSKSLQVTRIFLQALNLGIEVINTTDHLKFSKDCGRMLTRMWYCSYCQGLMMVKPCGGYCNVVMQGCMAGVVEIDKYWREYILSLEELVNGMYRIYDMENVLLGLFSTIHDSIQYVQKNAGKLTTTIGKLCAHSQQRQYRSAYYPEDLFIDKKVLKVAHVEHEETLSSRRRELIQKLKSFISFYSALPGYICSHSPVAENDTLCWNGQELVERYSQKAARNGMKNQFNLHELKMKGPEPVVSQIIDKLKHINQLLRTMSMPKGRVLDKNLDEEGFESGDCGDDEDECIGGSGDGMIKVKNQLRFLAELAYDLDVDDAPGNSQQATPKDNEISTFHNLGNVHS

SEQ ID NO: 462 - protein, 556 aa, Artificial Sequence
  Amino acids 25-580 of SEQ ID NO: 460 human GPC3 full-length (UNIPROT)
QPPPPPPDATCHQVRSFFQRLQPGLKWVPETPVPGSDLQVCLPKGPTCCSRKMEEKYQLTARLNMEQLLQSASMELKFLIIQNAAVFQEAFEIVVRHAKNYTNAMFKNNYPSLTPQAFEFVGEFFTDVSLYILGSDINVDDMVNELFDSLFPVIYTQLMNPGLPDSALDINECLRGARRDLKVFGNFPKLIMTQVSKSLQVTRIFLQALNLGIEVINTTDHLKFSKDCGRMLTRMWYCSYCQGLMMVKPCGGYCNVVMQGCMAGVVEIDKYWREYILSLEELVNGMYRIYDMENVLLGLFSTIHDSIQYVQKNAGKLTTTIGKLCAHSQQRQYRSAYYPEDLFIDKKVLKVAHVEHEETLSSRRRELIQKLKSFISFYSALPGYICSHSPVAENDTLCWNGQELVERYSQKAARNGMKNQFNLHELKMKGPEPVVSQIIDKLKHINQLLRTMSMPKGRVLDKNLDEEGFESGDCGDDEDECIGGSGDGMIKVKNQLRFLAELAYDLDVDDAPGNSQQATPKDNEISTFHNLGNVHSPLKLLTSMAISVVCFFFLVH

SEQ ID NO: 463 - protein, 536 aa, Artificial Sequence
  Amino acids 25-560 of SEQ ID NO: 460 human GPC3 full-length (UNIPROT)
QPPPPPPDATCHQVRSFFQRLQPGLKWVPETPVPGSDLQVCLPKGPTCCSRKMEEKYQLTARLNMEQLLQSASMELKFLIIQNAAVFQEAFEIVVRHAKNYTNAMFKNNYPSLTPQAFEFVGEFFTDVSLYILGSDINVDDMVNELFDSLFPVIYTQLMNPGLPDSALDINECLRGARRDLKVFGNFPKLIMTQVSKSLQVTRIFLQALNLGIEVINTTDHLKFSKDCGRMLTRMWYCSYCQGLMMVKPCGGYCNVVMQGCMAGVVEIDKYWREYILSLEELVNGMYRIYDMENVLLGLFSTIHDSIQYVQKNAGKLTTTIGKLCAHSQQRQYRSAYYPEDLFIDKKVLKVAHVEHEETLSSRRRELIQKLKSFISFYSALPGYICSHSPVAENDTLCWNGQELVERYSQKAARNGMKNQFNLHELKMKGPEPVVSQIIDKLKHINQLLRTMSMPKGRVLDKNLDEEGFESGDCGDDEDECIGGSGDGMIKVKNQLRFLAELAYDLDVDDAPGNSQQATPKDNEISTFHNLGNVHS

SEQ ID NO: 464 - protein, 334 aa, Artificial Sequence
  Amino acids 25-358 of SEQ ID NO: 460 human GPC3 full-length (UNIPROT)
QPPPPPPDATCHQVRSFFQRLQPGLKWVPETPVPGSDLQVCLPKGPTCCSRKMEEKYQLTARLNMEQLLQSASMELKFLIIQNAAVFQEAFEIVVRHAKNYTNAMFKNNYPSLTPQAFEFVGEFFTDVSLYILGSDINVDDMVNELFDSLFPVIYTQLMNPGLPDSALDINECLRGARRDLKVFGNFPKLIMTQVSKSLQVTRIFLQALNLGIEVINTTDHLKFSKDCGRMLTRMWYCSYCQGLMMVKPCGGYCNVVMQGCMAGVVEIDKYWREYILSLEELVNGMYRIYDMENVLLGLFSTIHDSIQYVQKNAGKLTTTIGKLCAHSQQRQYR

SEQ ID NO: 465 - protein, 202 aa, Artificial Sequence
  Amino acids 359-560 of SEQ ID NO: 460 human GPC3 full-length (UNIPROT)
SAYYPEDLFIDKKVLKVAHVEHEETLSSRRRELIQKLKSFISFYSALPGYICSHSPVAENDTLCWNGQELVERYSQKAARNGMKNQFNLHELKMKGPEPVVSQIIDKLKHINQLLRTMSMPKGRVLDKNLDEEGFESGDCGDDEDECIGGSGDGMIKVKNQLRFLAELAYDLDVDDAPGNSQQATPKDNEISTFHNLGNVHS

SEQ ID NO: 466 - protein, 222 aa, Artificial Sequence
  Amino acids 359-580 of SEQ ID NO: 460 human GPC3 full-length (UNIPROT)
SAYYPEDLFIDKKVLKVAHVEHEETLSSRRRELIQKLKSFISFYSALPGYICSHSPVAENDTLCWNGQELVERYSQKAARNGMKNQFNLHELKMKGPEPVVSQIIDKLKHINQLLRTMSMPKGRVLDKNLDEEGFESGDCGDDEDECIGGSGDGMIKVKNQLRFLAELAYDLDVDDAPGNSQQATPKDNEISTFHNLGNVHSPLKLLTSMAISVVCFFFLVH

SEQ ID NO: 467 - protein, 51 aa, Artificial Sequence
  Amino acids 510-560 of SEQ ID NO: 460 human GPC3 full-length (UNIPROT)
GDGMIKVKNQLRFLAELAYDLDVDDAPGNSQQATPKDNEISTFHNLGNVHS

SEQ ID NO: 468 - protein, 358 aa, Artificial Sequence
  Amino acids 1-358 of SEQ ID NO: 460 human GPC3 full-length (UNIPROT)
MAGTVRTACLVVAMLLSLDFPGQAQPPPPPPDATCHQVRSFFQRLQPGLKWVPETPVPGSDLQVCLPKGPTCCSRKMEEKYQLTARLNMEQLLQSASMELKFLIIQNAAVFQEAFEIVVRHAKNYTNAMFKNNYPSLTPQAFEFVGEFFTDVSLYILGSDINVDDMVNELFDSLFPVIYTQLMNPGLPDSALDINECLRGARRDLKVFGNFPKLIMTQVSKSLQVTRIFLQALNLGIEVINTTDHLKFSKDCGRMLTRMWYCSYCQGLMMVKPCGGYCNVVMQGCMAGVVEIDKYWREYILSLEELVNGMYRIYDMENVLLGLFSTIHDSIQYVQKNAGKLTTTIGKLCAHSQQRQYR

SEQ ID NO: 469 - protein, 2 aa, Artificial Sequence
  Linker amino acid sequence
  Variant (1)..(2): Can be in repeat of at least one and up to ten or more
GS

SEQ ID NO: 470 - protein, 5 aa, Artificial Sequence
  Linker amino acid sequence
  Variant (1)..(5): Can be in repeat of at least one and up to ten or more
GSGGS

SEQ ID NO: 471 - protein, 5 aa, Artificial Sequence
  Linker amino acid sequence
  Variant (1)..(5): Can be in repeat of at least one and up to ten or more
GGGGS

SEQ ID NO: 472 - protein, 4 aa, Artificial Sequence
  Linker amino acid sequence
  Variant (1)..(4): Can be in repeat of at least one and up to ten or more
GGGS

SEQ ID NO: 473 - protein, 21 aa, Artificial Sequence
  Linker amino acid sequence
SRGGGGSGGGGSGGGGSLEMA

SEQ ID NO: 474 - protein, 7 aa, Artificial Sequence
  Linker amino acid sequence
TSGGGGS

SEQ ID NO: 475 - protein, 22 aa, Artificial Sequence
  Linker amino acid sequence
AEAAAKEAAAKEAAAKEAAAKA

SEQ ID NO: 476 - protein, 6 aa, Artificial Sequence
  His-tag amino acid sequence
HHHHHH

SEQ ID NO: 477 - protein, 25 aa, Artificial Sequence
  His-tag and HA-tag amino acid sequence
TSGQAGQHHHHHHGAYPYDVPDYAS

SEQ ID NO: 478 - protein, 5 aa, Artificial Sequence
  Fc hinge amino acid sequence
CPPCP

SEQ ID NO: 479 - protein, 8 aa, Artificial Sequence
  Anti-CD3 antibody HC-CDR1 amino acid sequence
GYTFTRYT

SEQ ID NO: 480 - protein, 8 aa, Artificial Sequence
  Anti-CD3 antibody HC-CDR2 amino acid sequence
INPSRGYT

SEQ ID NO: 481 - protein, 12 aa, Artificial Sequence
  Anti-CD3 antibody HC-CDR3 amino acid sequence
ARYYDDHYCLDY

SEQ ID NO: 482 - protein, 5 aa, Artificial Sequence
  Anti-CD3 antibody LC-CDR1 amino acid sequence
QSVSY

SEQ ID NO: 483 - protein, 3 aa, Artificial Sequence
  Anti-CD3 antibody LC-CDR2 amino acid sequence
DTS

SEQ ID NO: 484 - protein, 9 aa, Artificial Sequence
  Anti-CD3 antibody LC-CDR3 amino acid sequence
QQWSSNPLT

SEQ ID NO: 485 - protein, 119 aa, Artificial Sequence
  Anti-CD3 antibody VH amino acid sequence
DVQLVQSGAEVKKPGASVKVSCKASGYTFTRYTMHWVRQAPGQGLEWIGYINPSRGYTNYADSVKGRFTITTDKSTSTAYMELSSLRSEDTATYYCARYYDDHYCLDYWGQGTTVTVSS

SEQ ID NO: 486 - protein, 106 aa, Artificial Sequence
  Anti-CD3 antibody VL amino acid sequence
DIVLTQSPATLSLSPGERATLSCRASQSVSYMNWYQQKPGKAPKRWIYDTSKVASGVPARFSGSGSGTDYSLTINSLEAEDAATYYCQQWSSNPLTFGGGTKVEIK

SEQ ID NO: 487 - protein, 243 aa, Artificial Sequence
  Anti-CD3 scFv amino acid sequence
DVQLVQSGAEVKKPGASVKVSCKASGYTFTRYTMHWVRQAPGQGLEWIGYINPSRGYTNYADSVKGRFTITTDKSTSTAYMELSSLRSEDTATYYCARYYDDHYCLDYWGQGTTVTVSSGEGTSTGSGGSGGSGGADDIVLTQSPATLSLSPGERATLSCRASQSVSYMNWYQQKPGKAPKRWIYDTSKVASGVPARFSGSGSGTDYSLTINSLEAEDAATYYCQQWSSNPLTFGGGTKVEIK

SEQ ID NO: 488 - protein, 498 aa, Artificial Sequence
  Anti-nGPC3 (GPC3A-034) scFv-anti-CD3 scFv amino acid sequence
QPVLTQPPSASGTPGQRVTISCSGSSSNIGSNNVIWYQQLPGAAPKLLIYSNHRRPSGVPDRFSGSRSGTSASLAISGLQSEDEADYYCAAWDDSLDGYLFGTGTKVTVLGSRGGGGSGGGGSGGGGSLEMAQVQLQQWGAGLLKPSETLSLTCAVYGGSFSGYYWSWIRQPPGKGLEWIGEINHSGSTNYNPSLKSRVTISVDTSKNQFSLELSSVTAADTAVYYCARGYGGRFDYWGQGTLVTVSSTSGGGGSDVQLVQSGAEVKKPGASVKVSCKASGYTFTRYTMHWVRQAPGQGLEWIGYINPSRGYTNYADSVKGRFTITTDKSTSTAYMELSSLRSEDTATYYCARYYDDHYCLDYWGQGTTVTVSSGEGTSTGSGGSGGSGGADDIVLTQSPATLSLSPGERATLSCRASQSVSYMNWYQQKPGKAPKRWIYDTSKVASGVPARFSGSGSGTDYSLTINSLEAEDAATYYCQQWSSNPLTFGGGTKVEIK

SEQ ID NO: 489 - protein, 497 aa, Artificial Sequence
  Anti-GPC3 (GPC3B-87) scFv-anti-CD3 scFv amino acid sequence
DVVMTQSPLSLPVTPGEPASVSCRSSQSLLHSNGYNYLDWYLQKPGQSPQLLIYLGSNRASGVPDRFSGSGSGTDFTLKISRVEAEDVGVYYCMQALQTPWTFGQGTKVEIKRSRGGGGSGGGGSGGGGSLEMAEVQLVQSGAEVRKPGSSVKVSCQASGGTFGSYAISWVRQAPGQGLEWMGRIIPVLGRTKYAQKFQGRVTVTADTSTSTVYMELTSLTSEDTAVYYCARTNDSWGQGTLVTVSSTSGGGGSDVQLVQSGAEVKKPGASVKVSCKASGYTFTRYTMHWVRQAPGQGLEWIGYINPSRGYTNYADSVKGRFTITTDKSTSTAYMELSSLRSEDTATYYCARYYDDHYCLDYWGQGTTVTVSSGEGTSTGSGGSGGSGGADDIVLTQSPATLSLSPGERATLSCRASQSVSYMNWYQQKPGKAPKRWIYDTSKVASGVPARFSGSGSGTDYSLTINSLEAEDAATYYCQQWSSNPLTFGGGTKVEIK

SEQ ID NO: 490 - protein, 18 aa, Artificial Sequence
  Linker amino acid sequence
GEGTSTGSGGSGGSGGAD

SEQ ID NO: 491 - protein, 470 aa, Artificial Sequence
  GPC3A-034 scFv-CAR amino acid sequence
QPVLTQPPSASGTPGQRVTISCSGSSSNIGSNNVIWYQQLPGAAPKLLIYSNHRRPSGVPDRFSGSRSGTSASLAISGLQSEDEADYYCAAWDDSLDGYLFGTGTKVTVLGSRGGGGSGGGGSGGGGSLEMAQVQLQQWGAGLLKPSETLSLTCAVYGGSFSGYYWSWIRQPPGKGLEWIGEINHSGSTNYNPSLKSRVTISVDTSKNQFSLELSSVTAADTAVYYCARGYGGRFDYWGQGTLVTVSSAAAIEVMYPPPYLDNEKSNGTIIHVKGKHLCPSPLFPGPSKPFWVLVVVGGVLACYSLLVTVAFIIFWVRSKRSRLLHSDYMNMTPRRPGPTRKHYQPYAPPRDFAAYRSRVKFSRSADAPAYQQGQNQLYNELNLGRREEYDVLDKRRGRDPEMGGKPRRKNPQEGLYNELQKDKMAEAYSEIGMKGERRRGKGHDGLYQGLSTATKDTYDALHMQALPPR

SEQ ID NO: 492 - protein, 287 aa, Artificial Sequence
  GPC3A-034 (VHCH)-TCR delta amino acid sequence
QVQLQQWGAGLLKPSETLSLTCAVYGGSFSGYYWSWIRQPPGKGLEWIGEINHSGSTNYNPSLKSRVTISVDTSKNQFSLELSSVTAADTAVYYCARGYGGRFDYWGQGTLVTVSSASTKGPSVFPLAPSSKSTSGGTAALGCLVKDYFPEPVTVSWNSGALTSGVHTFPAVLQSSGLYSLSSVVTVPSSSLGTQTYICNVNHKPSNTKVDKRVEPKSCEVKTDSTDHVKPKETENTKQPSKSCHKPKAIVHTEKVNMMSLTVLGLRMLFAKTVAVNFLLTAKLFFL

SEQ ID NO: 493 - protein, 283 aa, Artificial Sequence
  GPC3A-034 (VLCL)-TCR gamma amino acid sequence
QPVLTQPPSASGTPGQRVTISCSGSSSNIGSNNVIWYQQLPGAAPKLLIYSNHRRPSGVPDRFSGSRSGTSASLAISGLQSEDEADYYCAAWDDSLDGYLFGTGTKVTVLGQPKANPTVTLFPPSSEELQANKATLVCLISDFYPGAVTVAWKADGSPVKAGVETTKPSKQSNNKYAASSYLSLTPEQWKSHRSYSCQVTHEGSTVEKTVAPTECSPIKTDVITMDPKDNCSKDANDTLLLQLTNTSAYYMYLLLLLKSVVYFAIITCCLLRRTAFCCNGEKS

SEQ ID NO: 494 - protein, 219 aa, Artificial Sequence
  CD28-CD3 zeta CAR domain fusion amino acid sequence
IEVMYPPPYLDNEKSNGTIIHVKGKHLCPSPLFPGPSKPFWVLVVVGGVLACYSLLVTVAFIIFWVRSKRSRLLHSDYMNMTPRRPGPTRKHYQPYAPPRDFAAYRSRVKFSRSADAPAYQQGQNQLYNELNLGRREEYDVLDKRRGRDPEMGGKPRRKNPQEGLYNELQKDKMAEAYSEIGMKGERRRGKGHDGLYQGLSTATKDTYDALHMQALPPR

SEQ ID NO: 495 - protein, 68 aa, Artificial Sequence
  TCR delta chain amino acid sequence
EVKTDSTDHVKPKETENTKQPSKSCHKPKAIVHTEKVNMMSLTVLGLRMLFAKTVAVNFLLTAKLFFL

SEQ ID NO: 496 - protein, 67 aa, Artificial Sequence
  TCR gamma chain amino acid sequence
PIKTDVITMDPKDNCSKDANDTLLLQLTNTSAYYMYLLLLLKSVVYFAIITCCLLRRTAFCCNGEKS

SEQ ID NO: 497 - protein, 5 aa, Artificial Sequence
  GC33 antibody HC-CDR1 amino acid sequence
DYEMH

SEQ ID NO: 498 - protein, 17 aa, Artificial Sequence
  GC33 antibody HC-CDR2 amino acid sequence
ALDPKTGDTAYSQKFKG

SEQ ID NO: 499 - protein, 6 aa, Artificial Sequence
  GC33 antibody HC-CDR3 amino acid sequence
FYSYTY

SEQ ID NO: 500 - protein, 16 aa, Artificial Sequence
  GC33 antibody LC-CDR1 amino acid sequence
RSSQSLVHSNGNTYLH

SEQ ID NO: 501 - protein, 7 aa, Artificial Sequence
  GC33 antibody LC-CDR2 amino acid sequence
KVSNRFS

SEQ ID NO: 502 - protein, 9 aa, Artificial Sequence
  GC33 antibody LC-CDR3 amino acid sequence
SQNTHVPPT

SEQ ID NO: 503 - protein, 116 aa, Artificial Sequence
  GC33 antibody VH amino acid sequence
QVQLQQSGAELVKPGASVKLSCKASGYTFTDYEMHWVKQTPVHGLKWMIGALDPKTGDTAYSQKFKGKATLTADKSSSTAYMELRSLTSEDSAVYYCTRFYSYTYWGQGTLVTVSA

SEQ ID NO: 504 - protein, 112 aa, Artificial Sequence
  GC33 antibody VL amino acid sequence
DVVMTQTPLSLPVSLGDQASISCRSSQSLVHSNGNTYLHWYLQKPGQSPKLLIYKVSNRFSGVPDRFSGSGSGTDFTLKISRVEAEDLGVYFCSQNTHVPPTFGSGTKLEIK

SEQ ID NO: 505 - protein, 440 aa, Artificial Sequence
  GPC3A-039 mouse heavy chain amino acid sequence
QVQLVQSGGGLVHPGGSLRLSCAGSGFTFSSYAMHWVRQAPGKGLEWVSAIGTGGGTYYADSVKGRFTISRDNAKNSLYLQMNSLRAEDTAVYYCARYGRKSIDAWGQGTLVTVSSAKTTPPSVYPLAPGSAAQTNSMVTLGCLVKGYFPEPVTVTWNSGSLSSGVHTFPAVLQSDLYTLSSSVTVPSSTWPSETVTCNVAHPASSTKVDKKIVPRDCGCKPCICTVPEVSSVFIFPPKPKDVLTITLTPKVTCVVVAISKDDPEVQFSWFVDDVEVHTAQTQPREEQFNSTFRSVSELPIMHQDWLNGKEFKCRVNSAAFPAPIEKTISKTKGRPKAPQVYTIPPPKEQMAKDKVSLTCMITDFFPEDITVEWQWNGQPAENYKNTQPIMDTDGSYFVYSKLNVQKSNWEAGNTFTCSVLHEGLHNHHTEKSLSHSPGK

SEQ ID NO: 506 - protein, 214 aa, Artificial Sequence
  GPC3A-039 mouse light chain amino acid sequence
SYVLTQPPSVSVAPGKTARITCGGNNIGSKSVHWYQQKPGQAPVLVIYYDSDRPSGIPERFSGSNSGNTATLTISRVEAGDEADYYCQVWDSSSDHWVFGGGTKLTVLGQPKSSPSVTLFPPSSEELETNKATLVCTITDFYPGVVTVDWKVDGTPVTQGMETTQPSKQSNNKYMASSYLTLTARAWERHSSYSCQVTHEGHTVEKSLSRADCS

SEQ ID NO: 507 - protein, 324 aa, Artificial Sequence
  Mouse IgG1 heavy chain constant domain amino acid sequence
AKTTPPSVYPLAPGSAAQTNSMVTLGCLVKGYFPEPVTVTWNSGSLSSGVHTFPAVLQSDLYTLSSSVTVPSSTWPSETVTCNVAHPASSTKVDKKIVPRDCGCKPCICTVPEVSSVFIFPPKPKDVLTITLTPKVTCVVVAISKDDPEVQFSWFVDDVEVHTAQTQPREEQFNSTFRSVSELPIMHQDWLNGKEFKCRVNSAAFPAPIEKTISKTKGRPKAPQVYTIPPPKEQMAKDKVSLTCMITDFFPEDITVEWQWNGQPAENYKNTQPIMDTDGSYFVYSKLNVQKSNWEAGNTFTCSVLHEGLHNHHTEKSLSHSPGK

SEQ ID NO: 508 - protein, 105 aa, Artificial Sequence
  Mouse lambda light chain constant domain amino acid sequence
QPKSSPSVTLFPPSSEELETNKATLVCTITDFYPGVVTVDWKVDGTPVTQGMETTQPSKQSNNKYMASSYLTLTARAWERHSSYSCQVTHEGHTVEKSLSRADCS

SEQ ID NO: 509 - protein, 20 aa, Artificial Sequence
  Signal peptide amino acid sequence
METDTLLLWVLLLWVPGSTG

SEQ ID NO: 510 - protein, 228 aa, Artificial Sequence
  GC33 antibody amino acid sequence
QVQLQQSGAELVKPGASVKLSCKASGYTFTDYEMHWVKQTPVHGLKWMIGALDPKTGDTAYSQKFKGKATLTADKSSSTAYMELRSLTSEDSAVYYCTRFYSYTYWGQGTLVTVSADVVMTQTPLSLPVSLGDQASISCRSSQSLVHSNGNTYLHWYLQKPGQSPKLLIYKVSNRFSGVPDRFSGSGSGTDFTLKISRVEAEDLGVYFCSQNTHVPPTFGSGTKLEIK

SEQ ID NO: 511 - protein, 500 aa, Artificial Sequence
  Anti-nGPC3 (GPC3A-037) scFv-anti-CD3 scFv amino acid sequence
QSVLTQPPSVSAAPGQRVTISCSGTRSNIGSDYVSWYQHLPGTAPKLLVYGDNLRPSGIPDRFSASKSGTSATLGITGLQTGDEADYYCGTWDYTLNGVVFGGGTKLTVLGSRGGGGSGGGGSGGGGSLEMAQVQLVESGGGLVQPGGSLRLSCAASGFTFSSYAMSWVRQAPGKGLEWVSVIYSGGSSTYYADSVKGRFTISRDNSKNTLYLQMNSLRAEDTAVYYCARTSYLNHGDYWGQGTLVTVSSTSGGGGSDVQLVQSGAEVKKPGASVKVSCKASGYTFTRYTMHWVRQAPGQGLEWIGYINPSRGYTNYADSVKGRFTITTDKSTSTAYMELSSLRSEDTATYYCARYYDDHYCLDYWGQGTTVTVSSGEGTSTGSGGSGGSGGADDIVLTQSPATLSLSPGERATLSCRASQSVSYMNWYQQKPGKAPKRWIYDTSKVASGVPARFSGSGSGTDYSLTINSLEAEDAATYYCQQWSSNPLTFGGGTKVEIK

SEQ ID NO: 512 - protein, 498 aa, Artificial Sequence
  Anti-nGPC3 (GPC3A-045) scFv-anti-CD3 scFv amino acid sequence
QSVLTQPPSVSGTPGQRVIISCPGSTSNIGTNTVNWYQQFPGTAPKLLIYSNNQRPSGVPDRFSGSKSGTSASLAISGLQSEDEADYYCAAWDDSLNGVVFGGGTKLTVLGSRGGGGSGGGGSGGGGSLEMAQMQLVQSGGGLVKPGGSLRLSCAASGFTFSDYYMSWIRQAPGKGLEWVSYISSSGSTIYYADSVKGRFTISRDNAKNSLYLQMNSLRAEDTAVYYCARASDLYGDWGQGTLVTVSSTSGGGGSDVQLVQSGAEVKKPGASVKVSCKASGYTFTRYTMHWVRQAPGQGLEWIGYINPSRGYTNYADSVKGRFTITTDKSTSTAYMELSSLRSEDTATYYCARYYDDHYCLDYWGQGTTVTVSSGEGTSTGSGGSGGSGGADDIVLTQSPATLSLSPGERATLSCRASQSVSYMNWYQQKPGKAPKRWIYDTSKVASGVPARFSGSGSGTDYSLTINSLEAEDAATYYCQQWSSNPLTFGGGTKVEIK

SEQ ID NO: 513 - protein, 503 aa, Artificial Sequence
  Anti-nGPC3 (GPC3A-046) scFv-anti-CD3 scFv amino acid sequence
QAVLTQPPSVSGTPGQRVTISCSGSSSNFGSNTVHWYQQVPGTAPKLLIFSNTQRPSEIPDRFSGSKSGTSASLAISGLQSEDEADYYCAAWDDSLTGVVFGGGTKLTVLGSRGGGGSGGGGSGGGGSLEMAQVQLVQSGAEVKKPGASVTVSCKASGYRFSNYGVSWVRQAPGQGLEWMGWISGSNGNTNYAQKFLGRVTMTTDTSTTTAYMELSSLRSDDTAVYYCARGNRRYYSPIIDPWGQGTLVTVSSTSGGGGSDVQLVQSGAEVKKPGASVKVSCKASGYTFTRYTMHWVRQAPGQGLEWIGYINPSRGYTNYADSVKGRFTITTDKSTSTAYMELSSLRSEDTATYYCARYYDDHYCLDYWGQGTTVTVSSGEGTSTGSGGSGGSGGADDIVLTQSPATLSLSPGERATLSCRASQSVSYMNWYQQKPGKAPKRWIYDTSKVASGVPARFSGSGSGTDYSLTINSLEAEDAATYYCQQWSSNPLTFGGGTKVEIK

SEQ ID NO: 514 - protein, 497 aa, Artificial Sequence
  Anti-nGPC3 (GPC3A-055) scFv-anti-CD3 scFv amino acid sequence
QPVLTQPPSVSVAPGKTARITCGGNNIGSKSVHWYQQKPGQAPVLVIYYDSDRPSGIPERFSGSNSGNTATLTISRVEAGDEADYYCQVWDSSSDHYVFGTGTKVTVLGSRGGGGSGGGGSGGGGSLEMAQVQLVQSGAEVKKPGASVKVSCKASGYTFTSYYMHWVRQAPGQGLEWMGIINPSGGSTSYAQKFQGRVTMTRDTSTSTVYMELSSLRSEDTAVYYCARWHGGPYDYWGQGTLVTVSSTSGGGGSDVQLVQSGAEVKKPGASVKVSCKASGYTFTRYTMHWVRQAPGQGLEWIGYINPSRGYTNYADSVKGRFTITTDKSTSTAYMELSSLRSEDTATYYCARYYDDHYCLDYWGQGTTVTVSSGEGTSTGSGGSGGSGGADDIVLTQSPATLSLSPGERATLSCRASQSVSYMNWYQQKPGKAPKRWIYDTSKVASGVPARFSGSGSGTDYSLTINSLEAEDAATYYCQQWSSNPLTFGGGTKVEIK

SEQ ID NO: 515 - protein, 499 aa, Artificial Sequence
  Anti-nGPC3 (GPC3A-058) scFv-anti-CD3 scFv amino acid sequence
QSVLTQPPSVSVAPGKTARITCGGNNIGSKSVHWYQQKPGQAPVLVVYDDSDRPSGIPERFSGSNSGNTATLTISRVEAGDEADYYCQVWDSSSDHVFGTGTKVTVLGSRGGGGSGGGGSGGGGSLEMAQVQLVQSGADVRKPGASVKVSCKASGYTFASHGISWVRQAPGQGLEWLGWISPYTGNTNYAQKFQGRVTMATDTSTSTAYMELRSLRSDDTAIYYCARGKRTLASCFDYWGQGTLVTVSSTSGGGGSDVQLVQSGAEVKKPGASVKVSCKASGYTFTRYTMHWVRQAPGQGLEWIGYINPSRGYTNYADSVKGRFTITTDKSTSTAYMELSSLRSEDTATYYCARYYDDHYCLDYWGQGTTVTVSSGEGTSTGSGGSGGSGGADDIVLTQSPATLSLSPGERATLSCRASQSVSYMNWYQQKPGKAPKRWIYDTSKVASGVPARFSGSGSGTDYSLTINSLEAEDAATYYCQQWSSNPLTFGGGTKVEIK

SEQ ID NO: 516 - protein, 472 aa, Artificial Sequence
  ET230-37-28Z CAR amino acid sequence
QSVLTQPPSVSAAPGQRVTISCSGTRSNIGSDYVSWYQHLPGTAPKLLVYGDNLRPSGIPDRFSASKSGTSATLGITGLQTGDEADYYCGTWDYTLNGVVFGGGTKLTVLGSRGGGGSGGGGSGGGGSLEMAQVQLVESGGGLVQPGGSLRLSCAASGFTFSSYAMSWVRQAPGKGLEWVSVIYSGGSSTYYADSVKGRFTISRDNSKNTLYLQMNSLRAEDTAVYYCARTSYLNHGDYWGQGTLVTVSSAAAIEVMYPPPYLDNEKSNGTIIHVKGKHLCPSPLFPGPSKPFWVLVVVGGVLACYSLLVTVAFIIFWVRSKRSRLLHSDYMNMTPRRPGPTRKHYQPYAPPRDFAAYRSRVKFSRSADAPAYQQGQNQLYNELNLGRREEYDVLDKRRGRDPEMGGKPRRKNPQEGLYNELQKDKMAEAYSEIGMKGERRRGKGHDGLYQGLSTATKDTYDALHMQALPPR

SEQ ID NO: 517 - protein, 248 aa, Artificial Sequence; identical to SEQ ID NO: 419
  ET230-45-28Z CAR amino acid sequence

SEQ ID NO: 518 - protein, 253 aa, Artificial Sequence; identical to SEQ ID NO: 420
  ET230-46-28Z CAR amino acid sequence

SEQ ID NO: 519 - protein, 247 aa, Artificial Sequence; identical to SEQ ID NO: 429
  ET230-55-28Z CAR amino acid sequence

SEQ ID NO: 520 - protein, 249 aa, Artificial Sequence; identical to SEQ ID NO: 432
  ET230-58-28Z CAR amino acid sequence

SEQ ID NO: 521 - protein, 247 aa, Artificial Sequence; identical to SEQ ID NO: 452
  ET230-87-28Z CAR amino acid sequence

SEQ ID NO: 522 - protein, 288 aa, Artificial Sequence
  anti-AFP158/HLA-A*02:01-caTCR-6MD delta
EVQLVQSGAEVKKPGESLTISCKASGYSFPNYWITWVRQMSGGGLEWMGRIDPGDSYTTYNPSFQGHVTISIDKSTNTAYLHWNSLKASDTAMYYCARYYVSLVDIWGQGTLVTVSSASTKGPSVFPLAPSSKSTSGGTAALGCLVKDYFPEPVTVSWNSGALTSGVHTFPAVLQSSGLYSLSSVVTVPSSSLGTQTYICNVNHKPSNTKVDKRVEPKSCEVKTDSTDHVKPKETENTKQPSKSCHKPKAIVHTEKVNMMSLTVLGLRMLFAKTVAVNFLLTAKLFFL

SEQ ID NO: 523 - protein, 283 aa, Artificial Sequence
  anti-AFP158/HLA-A*02:01-caTCR-6MD gamma
QSVLTQPASVSGSPGQSITISCTGTSSDVGGYNYVSWYQQHPGKAPKLMIYDVNNRPSEVSNRFSGSKSGNTASLTISGLQAEDEADYYCSSYTTGSRAVFGGGTKLTVLGQPKANPTVTLFPPSSEELQANKATLVCLISDFYPGAVTVAWKADGSPVKAGVETTKPSKQSNNKYAASSYLSLTPEQWKSHRSYSCQVTHEGSTVEKTVAPTECSPIKTDVITMDPKDNCSKDANDTLLLQLTNTSAYYMYLLLLLKSVVYFAIITCCLLRRTAFCCNGEKS

SEQ ID NO: 524 - DNA, 180 bp, Artificial Sequence
  6NFAT response element
ggaggaaaaactgtttcatacagaaggcgtggaggaaaaactgtttcatacagaaggcgtggaggaaaaactgtttcatacagaaggcgtggaggaaaaactgtttcatacagaaggcgtggaggaaaaactgtttcatacagaaggcgtggaggaaaaactgtttcatacagaaggcgt

SEQ ID NO: 525 - DNA, 149 bp, Artificial Sequence
  TA promoter
gccgccccgactgcatctgcgtgttccaattcgccaatgacaagacgctgggcggggtttgtgtcatcatagaactaaagacatgcaaatatatttcttccggggacaccgccagcaaacgcgagcaacgggccacggggatgaagcag

SEQ ID NO: 526 - DNA, 335 bp, Artificial Sequence
  NFAT-derived promoter
ggaggaaaaactgtttcatacagaaggcgtggaggaaaaactgtttcatacagaaggcgtggaggaaaaactgtttcatacagaaggcgtggaggaaaaactgtttcatacagaaggcgtggaggaaaaactgtttcatacagaaggcgtggaggaaaaactgtttcatacagaaggcgtctcgaggccgccccgactgcatctgcgtgttccaattcgccaatgacaagacgctgggcggggtttgtgtcatcatagaactaaagacatgcaaatatatttcttccggggacaccgccagcaaacgcgagcaacgggccacggggatgaagcag

SEQ ID NO: 527 - DNA, 544 bp, Artificial Sequence
  EF1-alpha promoter
ggatctgcgatcgctccggtgcccgtcagtgggcagagcgcacatcgcccacagtccccgagaagttggggggaggggtcggcaattgaacgggtgcctagagaaggtggcgcggggtaaactgggaaagtgatgtcgtgtactggctccgcctttttcccgagggtgggggagaaccgtatataagtgcagtagtcgccgtgaacgttctttttcgcaacgggtttgccgccagaacacagctgaagcttcgaggggctcgcatctctccttcacgcgcccgccgccctacctgaggccgccatccacgccggttgagtcgcgttctgccgcctcccgcctgtggtgcctcctgaactgcgtccgccgtctaggtaagtttaaagctcaggtcgagaccgggcctttgtccggcgctcccttggagcctacctagactcagccggctctccacgctttgcctgaccctgcttgctcaactctacgtctttgtttcgttttctgttctgcgccgttacagatccaagctgtgaccggcgcctac

SEQ ID NO: 528 - protein, 117 aa, Artificial Sequence
  EF1-alpha promoter
EVQLVQSGAEVKKPGESLTISCKASGYSFPNYWITWVRQMSGGGLEWMGRIDPGDSYTTYNPSFQGHVTISIDKSTNTAYLHWNSLKASDTAMYYCARYYVSLVDIWGQGTLVTVSS

SEQ ID NO: 529 - protein, 110 aa, Artificial Sequence
  IgVL domain of anti-AFP antibody
QSVLTQPASVSGSPGQSITISCTGTSSDVGGYNYVSWYQQHPGKAPKLMIYDVNNRPSEVSNRFSGSKSGNTASLTISGLQAEDEADYYCSSYTTGSRAVFGGGTKLTVL

SEQ ID NO: 530 - protein, 110 aa, Artificial Sequence
  CSR1
AAAIEVMYPPPYLDNEKSNGTIIHVKGKHLCPSPLFPGPSKPFWVLVVVGGVLACYSLLVTVAFIIFWVRSKRSRLLHSDYMNMTPRRPGPTRKHYQPYAPPRDFAAYRS

SEQ ID NO: 531 - protein, 360 aa, Artificial Sequence
  Anti-GPC3 CSR
QSVLTQPPSVSAAPGQRVTISCSGTRSNIGSDYVSWYQHLPGTAPKLLVYGDNLRPSGIPDRFSASKSGTSATLGITGLQTGDEADYYCGTWDYTLNGVVFGGGTKLTVLGSRGGGGSGGGGSGGGGSLEMAQVQLVESGGGLVQPGGSLRLSCAASGFTFSSYAMSWVRQAPGKGLEWVSVIYSGGSSTYYADSVKGRFTISRDNSKNTLYLQMNSLRAEDTAVYYCARTSYLNHGDYWGQGTLVTVSSAAAIEVMYPPPYLDNEKSNGTIIHVKGKHLCPSPLFPGPSKPFWVLVVVGGVLACYSLLVTVAFIIFWVRSKRSRLLHSDYMNMTPRRPGPTRKHYQPYAPPRDFAAYRS

SEQ ID NO: 532 - protein, 288 aa, Artificial Sequence; identical to SEQ ID NO: 522
  anti-AFP158/HLA-A*02:01-caTCR-1-0 delta

SEQ ID NO: 533 - protein, 283 aa, Artificial Sequence; identical to SEQ ID NO: 523
  anti-AFP158/HLA-A*02:01-caTCR-1-0 gamma

SEQ ID NO: 534 - protein, 288 aa, Artificial Sequence
  anti-AFP158/HLA-A*02:01-caTCR-1-TM5 delta
EVQLVQSGAEVKKPGESLTISCKASGYSFPNYWITWVRQMSGGGLEWMGRIDPGDSYTTYNPSFQGHVTISIDKSTNTAYLHWNSLKASDTAMYYCARYYVSLVDIWGQGTLVTVSSASTKGPSVFPLAPSSKSTSGGTAALGCLVKDYFPEPVTVSWNSGALTSGVHTFPAVLQSSGLYSLSSVVTVPSSSLGTQTYICNVNHKPSNTKVDKRVEPKSCEVKTDSTDHVKPKETENTKQPSKSCHKPKAIVHTEKVNMMSLTVLGLRVLFAKTVAVNFLLTAKLFFL

SEQ ID NO: 535 - protein, 283 aa, Artificial Sequence
  anti-AFP158/HLA-A*02:01-caTCR-1-TM5 gamma
QSVLTQPASVSGSPGQSITISCTGTSSDVGGYNYVSWYQQHPGKAPKLMIYDVNNRPSEVSNRFSGSKSGNTASLTISGLQAEDEADYYCSSYTTGSRAVFGGGTKLTVLGQPKANPTVTLFPPSSEELQANKATLVCLISDFYPGAVTVAWKADGSPVKAGVETTKPSKQSNNKYAASSYLSLTPEQWKSHRSYSCQVTHEGSTVEKTVAPTECSPIKTDVITMDPKDNCSKDANDTLLLQLTNTSAYLVYLLLLLKSVVYFVIVTCCLLRRTAFCCNGEKS

SEQ ID NO: 536 - protein, 43 aa, Artificial Sequence
  GPC33 fragment
LAELAYDLDVDDAPGNSQQATPKDNEISTFHNLGNVHSPLKLL